European Patent Specification EP 4 077 695 B1, published July 24, 2024. Title: Method for the fermentative production of guanidinoacetic acid. Applicant: Evonik Operations GmbH. The sequence listing filed with the application follows.

SEQUENCE LISTING (57 sequences)

SEQ ID NO: 1 - DNA, 1146 bp, Moorea producens strain PAL-8-15-08-1
  CDS (1)..(1143): Genbank accession Number WP_070390602
atgtcggaaaaaattgttaattcctggaatgaatgggatgaattggaagaaatggtggtaggaattgcagactatgctagctttgaaccaaaagaaccagggaatcatccgaaattaagaaatcaaaatttagcggaaatcattcctttccccagtggacctaaagaccctaaagtccttgaaaaagctaatgaagaattaaatggactggcttatttattaaaagaccacgatgtgatagtaagaagacccgaaaaaattgattttactaaatctctaaaaacaccttactttgaagttgcaaatcaatactgtggagtctgtcctcgggatgtcatgattacctttgggaatgaaatcatggaagcgactatgtcgaagagagctagattttttgaatacttaccttaccggaaattggtctatgaatattggaataaagacgagcatatgatttggaatgctgcgcctaaaccgactatgcaggatagtatgtatctagagaatttctgggagctgtctttagaagaacgatttaagcgtatgcatgattttgaattttgtattacacaagatgaagtaatttttgatgcggctgactgtagcagattaggaaaggatatattagttcaggaatcgatgacaacaaatagaacaggaattcggtggttaaaaaagcacctagaaccaagaggatttcgggttcaccctgttcattttccccttgattttttcccctcacacattgactgtacgtttgttcctttgcgaccaggtcttattttgacaaaccctgaaagacctatacgggaagaggaggagaagatttttaaagagaatggctgggagttgatcacagttcctcaaccgacttgctcgaatgatgaaatgccaatgttttgccagtccagtaagtggttgtcaatgaatgttctgagtatatcaccgacaaaggttatctgtgaggaaagagaaaaacctctccaagaattgttggataagcatggatttgaggtttttcctttaccctttagacatgtctttgaatttggggggtcttttcattgtgcaacttgggatattcgccgaaaaggtgagtgtgaagattatttaccaaatttaaactatcaaccgatttgtggttaa

SEQ ID NO: 2 - protein, 381 aa, Moorea producens strain PAL-8-15-08-1
MSEKIVNSWNEWDELEEMVVGIADYASFEPKEPGNHPKLRNQNLAEIIPFPSGPKDPKVLEKANEELNGLAYLLKDHDVIVRRPEKIDFTKSLKTPYFEVANQYCGVCPRDVMITFGNEIMEATMSKRARFFEYLPYRKLVYEYWNKDEHMIWNAAPKPTMQDSMYLENFWELSLEERFKRMHDFEFCITQDEVIFDAADCSRLGKDILVQESMTTNRTGIRWLKKHLEPRGFRVHPVHFPLDFFPSHIDCTFVPLRPGLILTNPERPIREEEEKIFKENGWELITVPQPTCSNDEMPMFCQSSKWLSMNVLSISPTKVICEEREKPLQELLDKHGFEVFPLPFRHVFEFGGSFHCATWDIRRKGECEDYLPNLNYQPICG

SEQ ID NO: 3 - DNA, 1248 bp, synthetic DNA
  RBS (49)..(52): Shine-Dalgarno Sequence AGGA
  CDS (58)..(1200): open reading frame of optimized  AGAT_Mp; protein is identical to genbank accession number WP_070390602
cgtctctgtggataactgagcggataagttcctagtacgcgtgcgagcaggaagaacatgagcgagaaaattgtgaacagctggaatgaatgggatgaactggaagaaatggttgttggtattgcagattatgcaagctttgaaccgaaagaaccgggtaatcatccgaaactgcgtaatcagaatctggcagaaattattccgtttccgagcggtccgaaagatccgaaagttctggaaaaagcaaatgaagaactgaatggtctggcctatctgctgaaagatcatgatgttattgttcgccgtccggaaaaaatcgactttaccaaaagcctgaaaaccccgtatttcgaagttgccaatcagtattgtggtgtttgtccgcgtgatgttatgattacctttggcaacgaaattatggaagccaccatgagcaaacgtgcccgtttttttgaatatctgccgtatcgtaaactggtgtatgagtattggaacaaagatgagcatatgatctggaatgcagcaccgaaaccgaccatgcaggatagcatgtatctggaaaacttttgggaactgagcctggaagaacgttttaaacgtatgcacgattttgagttttgcatcacccaggatgaagtgatttttgatgcagcagattgtagccgtctgggtaaagatattctggttcaagaaagcatgaccaccaatcgtaccggtattcgttggctgaaaaaacatctggaaccgcgtggttttcgtgttcatccggttcattttccgctggatttttttccgagccatattgattgtacctttgttccgctgcgtccgggtctgattctgaccaatccggaacgtccgattcgtgaagaagaagagaaaatcttcaaagagaatggctgggagctgattaccgttccgcagccgacctgtagcaatgatgaaatgccgatgttttgtcagagcagcaaatggctgagcatgaatgttctgagcattagcccgaccaaagttatttgtgaagaacgtgaaaaaccgctgcaagaactgctggataaacatggttttgaagtgtttccgctgccgtttcgtcatgtttttgaatttggtggtagctttcattgtgccacctgggatattcgtcgtaaaggtgaatgtgaagattatctgccgaatctgaattatcagccgatttgtggttaataagacgtccgcgagggccgtgttgccggtttcttcagagagacg

SEQ ID NO: 4 - protein, 381 aa, synthetic DNA; identical to SEQ ID NO: 2

SEQ ID NO: 5 - DNA, 30 bp, synthetic oligonucleotide
ccgttaactgccgagacaatcgcataaagg

SEQ ID NO: 6 - DNA, 34 bp, synthetic oligonucleotide
ctcctaggctaatattcttacctcggctggttgg

SEQ ID NO: 7 - DNA, 27 bp, synthetic oligonucleotide
ccgttaacacggctggcaaggaactta

SEQ ID NO: 8 - DNA, 41 bp, synthetic oligonucleotide
gccctaggtcaatattacaggccataaactaatgcttatcg

SEQ ID NO: 9 - DNA, 46 bp, synthetic oligonucleotide
ggaaacagctatgacatgattacgcggttatcgcggaatccgtatg

SEQ ID NO: 10 - DNA, 25 bp, PsodcarAB-LA-R
ttaagcgttttgtgcaactccgtct

SEQ ID NO: 11 - DNA, 50 bp, synthetic oligonucleotide
agacggagttgcacaaaacgcttaaaccctacttagctgccaattattcc

SEQ ID NO: 12 - DNA, 50 bp, synthetic oligonucleotide
ggtaggtggtggtgtctttactcatgggtaaaaaatcctttcgtaggttt

SEQ ID NO: 13 - DNA, 25 bp, synthetic oligonucleotide
atgagtaaagacaccaccacctacc

SEQ ID NO: 14 - DNA, 46 bp, synthetic oligonucleotide
gttgtaaaacgacggccagtgccaccggtgatgtggttcttcactg

SEQ ID NO: 15 - DNA, 1176 bp, Cylindrospermopsis raciborskii AWT205
  CDS (1)..(1176): genbank accession number EU140798.1
atgcaaacaagaattgtaaatagctggaatgagtgggatgaactaaaggagatggttgtcgggattgcagatggtgcttattttgaaccaactgagccaggtaaccgccctgctttacgcgataagaacattgccaaaatgttctcttttcccaggggtccgaaaaagcaagaggtaacagagaaagctaatgaggagttgaatgggctggtagcgcttctagaatcacagggcgtaactgtacgccgcccagagaaacataactttggcctgtctgtgaagacaccattctttgaggtagagaatcaatattgtgcggtctgcccacgtgatgttatgatcacctttgggaacgaaattctcgaagcaactatgtcacggcggtcacgcttctttgagtatttaccctatcgcaaactagtctatgaatattggcataaagatccagatatgatctggaatgctgcgcctaaaccgactatgcaaaatgccatgtaccgcgaagatttctgggagtgtccgatggaagatcgatttgagagtatgcatgattttgagttctgcgtcacccaggatgaggtgatttttgacgcagcagactgtagccgctttggccgtgatatttttgtgcaggagtcaatgacgactaatcgtgcagggattcgctggctcaaacggcatttagagccgcgtcgcttccgcgtgcatgatattcacttcccactagatattttcccatcccacattgattgtacttttgtccccttagcacctggggttgtgttagtgaatccagatcgccccatcaaagagggtgaagagaaactcttcatggataacggttggcaattcatcgaagcacccctccccacttccaccgacgatgagatgcctatgttctgccagtccagtaagtggttggcgatgaatgtgttaagcatttcccccaagaaggtcatctgtgaagagcaagagcatccgcttcatgagttgctagataaacacggctttgaggtctatccaattccctttcgcaatgtctttgagtttggcggttcgctccattgtgccacctgggatatccatcgcacgggaacctgtgaggattacttccctaaactaaactatacgccggtaactgcatcaaccaatggcgtttctcgcttcatcatttag

SEQ ID NO: 16 - protein, 391 aa, Cylindrospermopsis raciborskii AWT205
MQTRIVNSWNEWDELKEMVVGIADGAYFEPTEPGNRPALRDKNIAKMFSFPRGPKKQEVTEKANEELNGLVALLESQGVTVRRPEKHNFGLSVKTPFFEVENQYCAVCPRDVMITFGNEILEATMSRRSRFFEYLPYRKLVYEYWHKDPDMIWNAAPKPTMQNAMYREDFWECPMEDRFESMHDFEFCVTQDEVIFDAADCSRFGRDIFVQESMTTNRAGIRWLKRHLEPRRFRVHDIHFPLDIFPSHIDCTFVPLAPGVVLVNPDRPIKEGEEKLFMDNGWQFIEAPLPTSTDDEMPMFCQSSKWLAMNVLSISPKKVICEEQEHPLHELLDKHGFEVYPIPFRNVFEFGGSLHCATWDIHRTGTCEDYFPKLNYTPVTASTNGVSRFII

SEQ ID NO: 17 - DNA, 1272 bp, Homo sapiens
  CDS (1)..(1272): codes for NP_001473.1
  transit_peptide (1)..(111): mitochondrial localisation signal peptide
atgctgcgggtgcggtgtctgcgcggcgggagccgcggcgccgaggcggtgcactacatcggatctcggcttggacgaaccttgacaggatgggtgcagcgaactttccagagcacccaggcagctacggcttcctcccggaactcctgtgcagctgacgacaaagccactgagcctctgcccaaggactgccctgtctcttcttacaacgaatgggaccccttagaggaagtgatagtgggcagagcagaaaacgcctgtgttccaccgttcaccatcgaggtgaaggccaacacatatgaaaagtactggccattttaccagaagcaaggagggcattattttcccaaagatcatttgaaaaaggctgttgctgaaattgaagaaatgtgcaatattttaaaaacggaaggagtgacagtaaggaggcctgaccccattgactggtcattgaagtataaaactcctgattttgagtctacgggtttatacagtgcaatgcctcgagacatcctgatagttgtgggcaatgagattatcgaggctcccatggcatggcgttcacgcttctttgagtaccgagcgtacaggtcaattatcaaagactacttccaccgtggcgccaagtggacaacagctcctaagcccacaatggctgatgagctttataaccaggattatcccatccactctgtagaagacagacacaaattggctgctcagggaaaatttgtgacaactgagtttgagccatgctttgatgctgctgacttcattcgagctggaagagatatttttgcacagagaagccaggttacaaactacctaggcattgaatggatgcgtaggcatcttgctccagactacagagtgcatatcatctcctttaaagatcccaatcccatgcatattgatgctaccttcaacatcattggacctggtattgtgctttccaaccctgaccgaccatgtcaccagattgatcttttcaagaaagcaggatggactatcattactcctccaacaccaatcatcccagacgatcatccactctggatgtcatccaaatggctttccatgaatgtcttaatgctagatgaaaaacgtgttatggtggatgccaatgaagttccaattcaaaagatgtttgaaaagctgggtatcactaccattaaagttaacattcgtaatgccaattccctgggaggaggcttccattgctggacctgcgatgtccggcgccgaggcaccttacagtcctacttggactga

SEQ ID NO: 18 - protein, 423 aa, Homo sapiens
MLRVRCLRGGSRGAEAVHYIGSRLGRTLTGWVQRTFQSTQAATASSRNSCAADDKATEPLPKDCPVSSYNEWDPLEEVIVGRAENACVPPFTIEVKANTYEKYWPFYQKQGGHYFPKDHLKKAVAEIEEMCNILKTEGVTVRRPDPIDWSLKYKTPDFESTGLYSAMPRDILIVVGNEIIEAPMAWRSRFFEYRAYRSIIKDYFHRGAKWTTAPKPTMADELYNQDYPIHSVEDRHKLAAQGKFVTTEFEPCFDAADFIRAGRDIFAQRSQVTNYLGIEWMRRHLAPDYRVHIISFKDPNPMHIDATFNIIGPGIVLSNPDRPCHQIDLFKKAGWTIITPPTPIIPDDHPLWMSSKWLSMNVLMLDEKRVMVDANEVPIQKMFEKLGITTIKVNIRNANSLGGGFHCWTCDVRRRGTLQSYLD

SEQ ID NO: 19 - protein, 7 aa, Escherichia coli
MTDVTIK

SEQ ID NO: 20 - protein, 375 aa, Homo sapiens
MTDVTIKATEPLPKDCPVSSYNEWDPLEEVIVGRAENACVPPFTIEVKANTYEKYWPFYQKQGGHYFPKDHLKKAVAEIEEMCNILKTEGVTVRRPDPIDWSLKYKTPDFESTGLYSAMPRDILIVVGNEIIEAPMAWRSRFFEYRAYRSIIKDYFHRGAKWTTAPKPTMADELYNQDYPIHSVEDRHKLAAQGKFVTTEFEPCFDAADFIRAGRDIFAQRSQVTNYLGIEWMRRHLAPDYRVHIISFKDPNPMHIDATFNIIGPGIVLSNPDRPCHQIDLFKKAGWTIITPPTPIIPDDHPLWMSSKWLSMNVLMLDEKRVMVDANEVPIQKMFEKLGITTIKVNIRNANSLGGGFHCWTCDVRRRGTLQSYLD

SEQ ID NO: 21 - protein, 423 aa, Rattus norvegicus
MLRVRCLRGGSRGAEAVHYIGSRLGGSLTGWVQRTFQSTQAATASSQNSCAAEDKATHPLPKDCPVSSYNEWDPLEEVIVGRAENACVPPFTVEVKANTYEKYWPFYQKNGGLYFPKDHLKKAVAEVEEMCNILSMEGVTVKRPDPIDWSLKYKTPDFESTGLYSAMPRDILMVVGNEIIEAPMAWRSRFFEYRAYRSIIKDYFHRGAKWTTAPKPTMADELYDQDYPIHSVEDRHKLAAQGKFVTTEFEPCFDAADFIRAGRDIFAQRSQVTNYLGIEWMRRHLAPDYRVHIISFKDPNPMHIDATFNIIGPGLVLSNPDRPCHQIDLFKKAGWTIVTPPTPVIPDDHPLWMSSKWLSMNVLMLDEKRVMVDANEVPIQKMFEKLGISTIKVNIRNANSLGGGFHCWTCDVRRRGTLQSYFD

SEQ ID NO: 22 - protein, 375 aa, Rattus norvegicus
MTDVTIKATHPLPKDCPVSSYNEWDPLEEVIVGRAENACVPPFTVEVKANTYEKYWPFYQKNGGLYFPKDHLKKAVAEVEEMCNILSMEGVTVKRPDPIDWSLKYKTPDFESTGLYSAMPRDILMVVGNEIIEAPMAWRSRFFEYRAYRSIIKDYFHRGAKWTTAPKPTMADELYDQDYPIHSVEDRHKLAAQGKFVTTEFEPCFDAADFIRAGRDIFAQRSQVTNYLGIEWMRRHLAPDYRVHIISFKDPNPMHIDATFNIIGPGLVLSNPDRPCHQIDLFKKAGWTIVTPPTPVIPDDHPLWMSSKWLSMNVLMLDEKRVMVDANEVPIQKMFEKLGISTIKVNIRNANSLGGGFHCWTCDVRRRGTLQSYFD

SEQ ID NO: 23 - protein, 423 aa, Galeopterus variegatus; identical to SEQ ID NO: 21

SEQ ID NO: 24 - protein, 375 aa, Galeopterus variegatus
MTDVTIKATDPLPKDCPVSSYNEWDPLEEVIVGRAENACVPPFTVEVKANTYEKYWPFYQKHGGHYFPKDHLKKAVAEIEEMCNILKMEGVTVRRPDPIDWSLKYKTPDFESTGLYGAMPRDILIVVGNEIIEAPMAWRARFFEYRAYRSIIKDYFHRGAKWTTAPKPTMANELYDQDYPIYTVEDRHKLAAQGKFVTTEFEPCFDAADFIRAGRDIFAQRSQVTNYLGIEWMRRHLAPDYRVHIVSFKDPNPMHIDATFNIIGPGLVLSNPDRPCHQIDLFKKAGWTIITPPIPVIPDDHPLWMSSKWLSMNVLMLDEKRVMVDANEVPIQKMFGKLGISTIKVNIRNANSLGGGFHCWTCDVRRRGTLQSYFD

SEQ ID NO: 25 - DNA, 1278 bp, Cylindrospermopsis raciborskii AWT205
  RBS (49)..(52): Shine-Dalgarno-Sequence
  CDS (58)..(1230)
cgtctctgtggataactgagcggataagttcctagtacgcgtgcgagcaggaagaacatgcagacccgtattgttaatagctggaatgaatgggatgagctgaaagaaatggttgttggtattgcagatggtgcctattttgaaccgaccgaaccgggtaatcgtccggcactgcgtgataaaaacattgcaaaaatgtttagctttccgcgtggtccgaaaaaacaagaagttaccgaaaaagccaacgaagaactgaatggtctggttgcactgctggaaagccagggtgttaccgttcgtcgtccggaaaaacacaattttggtctgagcgttaaaaccccgttttttgaagtggaaaatcagtattgtgcagtgtgtccgcgtgatgttatgattacctttggtaacgaaattctggaagcaaccatgagccgtcgtagccgtttttttgaatatctgccgtatcgtaaactggtgtatgagtattggcataaagatccggatatgatttggaatgcagcaccgaaaccgaccatgcagaatgcaatgtatcgtgaagatttttgggaatgcccgatggaagatcgttttgaaagcatgcacgattttgaattttgcgtgacccaggatgaagtgatttttgatgcagcagattgcagccgttttggtcgtgatatttttgttcaagaaagcatgaccaccaatcgtgcaggtattcgctggctgaaacgtcatctggaaccgcgtcgttttcgtgttcatgatattcattttccgctggatatttttccgagccatattgattgtacctttgttccgctggcaccgggtgttgttctggttaatccggatcgtccgattaaagaaggtgaagaaaaactgtttatggacaacggctggcagtttattgaagcaccgctgccgaccagcaccgatgatgaaatgccgatgttttgtcagagcagcaaatggctggccatgaatgttctgagcattagcccgaaaaaagtgatctgtgaagaacaagaacatccgctgcatgaactgctggataaacatggttttgaggtttatccgattccgtttcgcaacgtgtttgaatttggtggtagcctgcattgtgcaacctgggatattcatcgtaccggcacctgtgaagattattttccgaaactgaattatacaccggttaccgcaagcaccaatggtgtgagccgttttatcatttaataagacgtccgcgagggccgtgttgccggtttcttcagagagacg

SEQ ID NO: 26 - protein, 391 aa, Cylindrospermopsis raciborskii AWT205; identical to SEQ ID NO: 16

SEQ ID NO: 27 - DNA, 1313 bp, Homo sapiens
  RBS (55)..(58): Shine-Dalgarno-Sequence
  CDS (62)..(1189)
ggtctcaagatatgaccatgattacgccaagcttgcatgcctgcaggaaaggagaggattgatgacagatgtaacgattaaagcgacggagccgctgccgaaggattgcccggttagctcttataatgagtgggatccgttggaggaggttatcgtgggccgcgcggagaacgcctgtgttcctccattcactatcgaggtgaaggccaacacttatgaaaagtactggccgttctaccagaagcaaggaggtcattacttccctaaggatcatctgaaaaaagcggtagccgaaattgaggagatgtgcaacatcctgaaaacggaaggcgtgaccgtccgtcgcccggatcccattgactggtcattgaagtataaaaccccggacttcgaaagcacgggtctttattcagccatgccgcgtgatatcctgatcgttgttggtaatgaaattattgaagcccctatggcctggcggagccgcttcttcgagtaccgtgcttatcggtctattatcaaagattacttccatcgtggtgcaaaatggacgactgctcctaagccaaccatggcagacgagttgtacaaccaggattaccctatccattcagtcgaagaccgccacaagctggcagcacagggtaaatttgtcacgactgagttcgaaccctgcttcgatgctgccgactttattcgtgccggacgggatattttcgcacaacgctcgcaagtaactaactacctcggcattgagtggatgcgtcggcatctggcccctgattaccgtgtccacatcattagcttcaaagacccgaacccgatgcacattgacgcgacttttaatatcatcggacccggtattgtgctgtcgaatcctgaccgcccgtgtcaccagattgacctttttaagaaagctggatggacgattatcacccctccaactccgattatccctgatgaccacccactctggatgtcctctaaatggctttccatgaacgttctgatgcttgacgagaagcgggttatggttgacgccaacgaagtccccattcagaaaatgtttgaaaagcttggcatcactacgattaaggtcaatatccgtaacgcgaacagcttgggcggtggttttcattgctggacgtgcgatgtgcgccgccggggaacccttcagtcctatctcgactaataagacgtctaaaaaaaaaccccgcccctgacagggcggggttttttttagtcgactctagaggatccccgggtaccgagctcgaattcactggccgtcgttttacagccaagcttgggagacc

SEQ ID NO: 28 - protein, 375 aa, Homo sapiens; identical to SEQ ID NO: 20

SEQ ID NO: 29 - DNA, 1313 bp, Rattus norvegicus
  RBS (55)..(58)
  CDS (62)..(1189)
ggtctcaagatatgaccatgattacgccaagcttgcatgcctgcaggaaaggagaggattgatgacagatgtaacgattaaagctactcatccgcttcctaaagattgccctgtgtcaagctataacgaatgggaccctttggaggaggtgatcgtgggccgtgctgagaacgcttgtgtacccccctttactgtcgaagtaaaagccaacacttacgagaagtactggccgttttaccagaaaaatggtggcctttatttccccaaagatcacctgaagaaagccgttgcagaggtcgaagagatgtgcaatattctgagcatggaaggtgtgactgtgaaacgcccagatccgattgactggtcacttaagtataagacgcccgactttgagtcgactggactttacagcgcgatgccgcgcgacattctgatggtagtgggaaatgagatcattgaggcgcccatggcgtggcggtcccgcttttttgagtatcgcgcgtaccggtcgattatcaaggattactttcaccggggcgcgaagtggaccaccgctccaaagcctacgatggctgacgagctttacgatcaagattaccccattcattcggttgaagaccgtcacaaattggcggcacaaggaaaattcgttacgactgagttcgagccttgctttgacgccgccgattttattcgggctggccgcgacatcttcgcacagcgttcacaagtaaccaactacttgggaatcgagtggatgcgtcggcaccttgccccagattaccgggtccatatcatttcatttaaagatcccaacccgatgcacattgacgctaccttcaatattattggaccaggactggtactctcaaaccctgatcggccctgtcaccagattgatctcttcaagaaggctggttggacgattgtcacgccaccgactcctgtaatcccggatgatcatcccctctggatgtcttccaaatggctctctatgaacgtactgatgctcgatgaaaaacgcgtgatggtagatgcgaatgaggtcccaattcaaaaaatgttcgagaagctgggcatctctactattaaggtgaacattcggaatgcaaactcgctcggaggaggtttccactgttggacttgtgacgtacggcggcgtggaactctccagagctacttcgattaataagacgtctaaaaaaaaaccccgcccctgacagggcggggttttttttagtcgactctagaggatccccgggtaccgagctcgaattcactggccgtcgttttacagccaagcttgggagacc

SEQ ID NO: 30 - protein, 375 aa, Rattus norvegicus; identical to SEQ ID NO: 22

SEQ ID NO: 31 - DNA, 1313 bp, Galeopterus variegatus
  RBS (55)..(58)
  CDS (62)..(1189)
ggtctcaagatatgaccatgattacgccaagcttgcatgcctgcaggaaaggagaggattgatgacagatgtaacgattaaagcgaccgatcctttgcctaaagattgccccgtgtcctcgtataatgaatgggacccgctcgaggaggtaatcgttggtcgggctgaaaatgcctgcgttccgcccttcactgttgaagtcaaagcgaatacttatgaaaagtactggccgttctatcaaaaacacggtggccactatttcccgaaagaccacctgaaaaaagctgttgctgagattgaagaaatgtgtaacatcctgaagatggaaggcgttacggttcgtcggccagacccaatcgattggtcactgaagtacaagacccccgactttgagtcgactggactctacggagctatgccccgtgatatcctcatcgttgttggcaatgaaatcatcgaagcccctatggcctggcgggcacgcttcttcgaataccgggcttatcgcagcatcatcaaggattattttcaccggggagccaaatggaccacggccccgaaacccactatggctaacgagttgtatgatcaagactatccgatctatacggtcgaggaccggcataaacttgcagcgcaaggtaaatttgtgactacggagttcgaaccttgtttcgatgccgctgattttattcgtgcaggacgcgatatctttgcgcaacggagccaagtaactaattacctcggtatcgagtggatgcggcgtcatctggcaccagattaccgtgttcacatcgtttcgttcaaagatccgaacccgatgcacattgatgccaccttcaacatcattggtcccggcctcgtgctcagcaatccagaccggccttgccaccaaattgacttgttcaaaaaagctggttggaccattattactcctccaattcccgtgattccagacgaccacccgctttggatgagctcaaaatggttgagcatgaatgtccttatgcttgatgagaagcgtgtcatggttgatgctaacgaggtaccaatccaaaagatgttcggcaagctgggtatttcaacgatcaaagtcaacattcggaacgccaattcactgggcggtggctttcactgctggacttgtgatgttcgtcggcggggcacgcttcaaagctatttcgactaataagacgtctaaaaaaaaaccccgcccctgacagggcggggttttttttagtcgactctagaggatccccgggtaccgagctcgaattcactggccgtcgttttacagccaagcttgggagacc

SEQ ID NO: 32 - protein, 375 aa, Galeopterus variegatus; identical to SEQ ID NO: 24

SEQ ID NO: 33 - DNA, 1211 bp, Synthetic DNA
tctagagatccgcgggggcccaggaggggggatctggcatttttgggaggtgtgaaatgagtgagaagatcgtcaactcgtggaacgaatgggatgagctcgaggagatggtggtcggcattgcggactatgccagcttcgaaccgaaagagccaggcaaccatcccaaactgcgcaaccagaacctggccgaaatcatccccttcccaagcggcccaaaggacccgaaggtgctggagaaagcgaacgaagagctgaatgggctggcttacctgctgaaggaccacgatgtgatcgtgcgtcgtcccgagaagatcgacttcaccaagagcctgaaaaccccgtatttcgaggttgccaaccagtactgcggcgtttgtcctcgcgacgtgatgatcacgtttggcaacgaaatcatggaagcgaccatgtccaaacgtgcacgcttcttcgaatacctcccctatcggaagctggtctacgagtactggaacaaggacgagcacatgatctggaacgcagccccgaaaccgaccatgcaggatagcatgtacctggaaaacttctgggagctctcgctggaagaacgcttcaagcggatgcacgacttcgaattctgcatcacccaagacgaggtgatcttcgatgccgccgattgctcccgcttgggtaaggacatcctggtgcaggaaagcatgaccaccaatcgcactggcatccgctggctgaagaagcatctcgaaccacgcggctttcgcgtccatccggtgcacttcccgttggacttcttccctagccacatcgactgcacgttcgtaccgttgcgtccgggtctgatcctgaccaatccggaacgcccgattcgcgaggaagaggagaagatcttcaaggagaatggctgggagctgatcaccgtaccgcagcctacctgctcgaacgacgagatgcccatgttctgccagagctcgaaatggctgtccatgaacgtcctgagcattagtcccaccaaggtgatctgcgaagaacgggaaaagccgctgcaagaactgctggacaagcacgggttcgaagtctttcccttgcctttccgccatgtgtttgagttcggtggcagctttcactgtgccacgtgggatattcgccgcaagggcgagtgcgaggactacctgccgaacctgaactaccagccgatttgcggctgacgcggatcc

SEQ ID NO: 34 - DNA, 2028 bp, Escherichia coli
ttaatctttctgcgaattgagatgacgccactggctgggcgtcatcccggtttcccgggtaaacaccaccgaaaaatagttactatcttcaaagccacattcggtcgaaatatcactgattaacaggcggctatgctggagaagatattgcgcatgacacactctgacctgtcgcagatattgattgatggtcattccagtctgctggcgaaattgctgacgcaaaacgcgctcactgcacgatgcctcatcacaaaatttatccagcgcaaagggacttttcaggctagccgccagccgggtaatcagcttatccagcaacgtttcgctggatgttggcggcaacgaatcactggtgtaacgatggcgattcagcaacatcaccaactgcccgaacagcaactcagccatttcgttagcaaacggcacatgctgactactttcatgctcaagctgaccgataacctgccgcgcctgcgccatccccatgctacctaagcgccagtgtggttgccctgcgctggcgttaaatcccggaatcgccccctgccagtcaagattcagcttcagacgctccgggcaataaataatattctgcaaaaccagatcgttaacggaagcgtaggagtgtttatcgtcagcatgaatgtaaaagagatcgccacgggtaatgcgataagggcgatcgttgagtacatgcaggccattaccgcgccagacaatcaccagctcacaaaaatcatgtgtatgttcagcaaagacatcttgcggataacggtcagccacagcgactgcctgctggtcgctggcaaaaaaatcatctttgagaagttttaactgatgcgccaccgtggctacctcggccagagaacgaagttgattattcgcaatatggcgtacaaatacgttgagaagattcgcgttattgcagaaagccatcccgtccctggcgaatatcacgcggtgaccagttaaactctcggcgaaaaagcgtcgaaaagtggttactgtcgctgaatccacagcgataggcgatgtcagtaacgctggcctcgctgtggcgtagcagatgtcgggctttcatcagtcgcaggcggttcaggtatcgctgaggcgtcagtcccgtttgctgcttaagctgccgatgtagcgtacgcagtgaaagagaaaattgatccgccacggcatcccaattcacctcatcggcaaaatggtcctccagccaggccagaagcaagttgagacgtgatgcgctgttttccaggttctcctgcaaactgcttttacgcagcaagagcagtaattgcataaacaagatctcgcgactggcggtcgagggtaaatcattttccccttcctgctgttccatctgtgcaaccagctgtcgcacctgctgcaatacgctgtggttaacgcgccagtgagacggatactgcccatccagctcttgtggcagcaactgattcagcccggcgagaaactgaaatcgatccggcgagcgatacagcacattggtcagacacagattatcggtatgttcatacagatgccgatcatgatcgcgtacgaaacagaccgtgccaccggtgatggtatagggctgcccattaaacacatgaatacccgtgccatgttcgacaatcacaatttcatgaaaatcatgatgatgttcaggaaaatccgcctgcgggagccggggttctatcgccacggacgcgttaccagacggaaaaaaatccacactatgtaatacggtcatactggcctcctgatgtcgtcaacacggcgaaatagtaatcacgaggtcaggttcttaccttaaattttcgacggaaaaccacgtaaaaaacgtcgatttttcaagatacagcgtgaattttcaggaaatgcggtgagcatcacatcaccacaattcagcaaattgtgaacatcatcacgttcatctttccctggttgccaatggcccattttcctgtcagtaacgagaaggtcgcgaattcaggcgctttttagactggtcgtaatgaa

SEQ ID NO: 35 - DNA, 107 bp, Escherichia coli
caaataaaacgaaaggctcagtcgaaagactgggcctttcgttttatctgttgtttgtcggtgaacgctctcctgagtaggacaaatccgccgggagcggatttgaa

SEQ ID NO: 36 - DNA, 24 bp, synthetic oligonucleotide
tctagagatccgcgggggcccagg

SEQ ID NO: 37 - DNA, 46 bp, synthetic oligonucleotide
agttccctactctcgcgtgctcgagggatccgcgtcagccgcaaat

SEQ ID NO: 38 - DNA, 10235 bp, various
tcaggcgggcaagaatgtgaataaaggccggataaaacttgtgcttatttttctttacggtctttaaaaaggccgtaatatccagctgaacggtctggttataggtacattgagcaactgactgaaatgcctcaaaatgttctttacgatgccattgggatatatcaacggtggtatatccagtgatttttttctccattttagcttccttagctcctgaaaatctcgataactcaaaaaatacgcccggtagtgatcttatttcattatggtgaaagttggaacctcttacgtgccgatcaacgtctcattttcgccaaaagttggcccagggcttcccggtatcaacagggacaccaggatttatttattctgcgaagtgatcttccgtcacaggtatttattcggcgcaaagtgcgtcgggtgatgctgccaacttactgatttagtgtatgatggtgtttttgaggtgctccagtggcttctgtttctatcagctgtccctcctgttcagctactgacggggtggtgcgtaacggcaaaagcaccgccggacatcagcgctagcggagtgtatactggcttactatgttggcactgatgagggtgtcagtgaagtgcttcatgtggcaggagaaaaaaggctgcaccggtgcgtcagcagaatatgtgatacaggatatattccgcttcctcgctcactgactcgctacgctcggtcgttcgactgcggcgagcggaaatggcttacgaacggggcggagatttcctggaagatgccaggaagatacttaacagggaagtgagagggccgcggcaaagccgtttttccataggctccgcccccctgacaagcatcacgaaatctgacgctcaaatcagtggtggcgaaacccgacaggactataaagataccaggcgtttccccctggcggctccctcgtgcgctctcctgttcctgcctttcggtttaccggtgtcattccgctgttatggccgcgtttgtctcattccacgcctgacactcagttccgggtaggcagttcgctccaagctggactgtatgcacgaaccccccgttcagtccgaccgctgcgccttatccggtaactatcgtcttgagtccaacccggaaagacatgcaaaagcaccactggcagcagccactggtaattgatttagaggagttagtcttgaagtcatgcgccggttaaggctaaactgaaaggacaagttttggtgactgcgctcctccaagccagttacctcggttcaaagagttggtagctcagagaaccttcgaaaaaccgccctgcaaggcggttttttcgttttcagagcaagagattacgcgcagaccaaaacgatctcaagaagatcatcttattaatcagataaaatatttctagatttcagtgcaatttatctcttcaaatgtagcacctgaagtcagccccatacgatataagttgtaattctcatgtttgacagcttatcatcgataagctttaatgcggtagtttatcacagttaaattgctaacgcagtcaggcaccgtgtatgaaatctaacaatgcgctcatcgtcatcctcggcaccgtcaccctggatgctgtaggcataggcttggttatgccggtactgccgggcctcttgcgggatatcgtccattccgacagcatcgccagtcactatggcgtgctgctagcgctatatgcgttgatgcaatttctatgcgcacccgttctcggagcactgtccgaccgctttggccgccgcccagtcctgctcgcttcgctacttggagccactatcgactacgcgatcatggcgaccacacccgtcctgtggatcctctacgccggacgcatcgtggccggcatcaccggcgccacaggtgcggttgctggcgcctatatcgccgacatcaccgatggggaagatcgggctcgccacttcgggctcatgagcgcttgtttcggcgtgggtatggtggcaggccccgtggccgggggactgttgggcgccatctccttgcatgcaccattccttgcggcggcggtgctcaacggcctcaacctactactgggctgcttcctaatgcaggagtcgcataagggagagcgtcgaccgatgcccttgagagccttcaacccagtcagctccttccggtgggcgcggggcatgactatcgtcgccgcacttatgactgtcttctttatcatgcaactcgtaggacaggtgccggcagcgctctgggtcattttcggcgaggaccgctttcgctggagcgcgacgatgatcggcctgtcgcttgcggtattcggaatcttgcacgccctcgctcaagccttcgtcactggtcccgccaccaaacgtttcggcgagaagcaggccattatcgccggcatggcggccgacgcgctgggctacgtcttgctggcgttcgcgacgcgaggctggatggccttccccattatgattcttctcgcttccggcggcatcgggatgcccgcgttgcaggccatgctgtccaggcaggtagatgacgaccatcagggacagcttcaaggatcgctcgcggctcttaccagcctaacttcgatcattggaccgctgatcgtcacggcgatttatgccgcctcggcgagcacatggaacgggttggcatggattgtaggcgccgccctataccttgtctgcctccccgcgttgcgtcgcggtgcatggagccgggccacctcgacctgaatggaagccggcggcacctcgctaacggattcaccactccaagaattggagccaatcaattcttgcggagaactgtgaatgcgcaaaccaacccttggcagaacatatccatcgcgtccgccatctccagcagccgcacgcggcgcatctcgggcagcgttgggtcctggccacgggtgcgcatgatcgtgctcctgtcgttgaggacccggctaggctggcggggttgccttactggttagcagaatgaatcaccgatacgcgagcgaacgtgaagcgactgctgctgcaaaacgtctgcgacctgagcaacaacatgaatggtcttcggtttccgtgtttcgtaaagtctggaaacgcggaagtcccctacgtgctgctgaagttgcccgcaacagagagtggaaccaaccggtgataccacgatactatgactgagagtcaacgccatgagcggcctcatttcttattctgagttacaacagtccgcaccgctgtccggtagctccttccggtgggcgcggggcatgactatcgtcgccgcacttatgactgtcttctttatcatgcaactcgtaggacaggtgccggcagcgcccaacagtcccccggccacggggcctgccaccatacccacgccgaaacaagcgccctgcaccattatgttccggatctgcatcgcaggatgctgctggctaccctgtggaacacctacatctgtattaacgaagcgctaaccgtttttatcaggctctgggaggcagaataaatgatcatatcgtcaattattacctccacggggagagcctgagcaaactggcctcaggcatttgagaagcacacggtcacactgcttccggtagtcaataaaccggtaaaccagcaatagacataagcggctatttaacgaccctgccctgaaccgacgaccgggtcgaatttgctttcgaatttctgccattcatccgcttattatcacttattcaggcgtagcaccaggcgtttaagggcaccaataactgccttaaaaaaattacgccccgccctgccactcatcgcagtactgttgtaattcattaagcattctgccgacatggaagccatcacaaacggcatgatgaacctgaatcgccagcggcatcagcaccttgtcgccttgcgtataatatttgcccatggatttaaatttaatctttctgcgaattgagatgacgccactggctgggcgtcatcccggtttcccgggtaaacaccaccgaaaaatagttactatcttcaaagccacattcggtcgaaatatcactgattaacaggcggctatgctggagaagatattgcgcatgacacactctgacctgtcgcagatattgattgatggtcattccagtctgctggcgaaattgctgacgcaaaacgcgctcactgcacgatgcctcatcacaaaatttatccagcgcaaagggacttttcaggctagccgccagccgggtaatcagcttatccagcaacgtttcgctggatgttggcggcaacgaatcactggtgtaacgatggcgattcagcaacatcaccaactgcccgaacagcaactcagccatttcgttagcaaacggcacatgctgactactttcatgctcaagctgaccgataacctgccgcgcctgcgccatccccatgctacctaagcgccagtgtggttgccctgcgctggcgttaaatcccggaatcgccccctgccagtcaagattcagcttcagacgctccgggcaataaataatattctgcaaaaccagatcgttaacggaagcgtaggagtgtttatcgtcagcatgaatgtaaaagagatcgccacgggtaatgcgataagggcgatcgttgagtacatgcaggccattaccgcgccagacaatcaccagctcacaaaaatcatgtgtatgttcagcaaagacatcttgcggataacggtcagccacagcgactgcctgctggtcgctggcaaaaaaatcatctttgagaagttttaactgatgcgccaccgtggctacctcggccagagaacgaagttgattattcgcaatatggcgtacaaatacgttgagaagattcgcgttattgcagaaagccatcccgtccctggcgaatatcacgcggtgaccagttaaactctcggcgaaaaagcgtcgaaaagtggttactgtcgctgaatccacagcgataggcgatgtcagtaacgctggcctcgctgtggcgtagcagatgtcgggctttcatcagtcgcaggcggttcaggtatcgctgaggcgtcagtcccgtttgctgcttaagctgccgatgtagcgtacgcagtgaaagagaaaattgatccgccacggcatcccaattcacctcatcggcaaaatggtcctccagccaggccagaagcaagttgagacgtgatgcgctgttttccaggttctcctgcaaactgcttttacgcagcaagagcagtaattgcataaacaagatctcgcgactggcggtcgagggtaaatcattttccccttcctgctgttccatctgtgcaaccagctgtcgcacctgctgcaatacgctgtggttaacgcgccagtgagacggatactgcccatccagctcttgtggcagcaactgattcagcccggcgagaaactgaaatcgatccggcgagcgatacagcacattggtcagacacagattatcggtatgttcatacagatgccgatcatgatcgcgtacgaaacagaccgtgccaccggtgatggtatagggctgcccattaaacacatgaatacccgtgccatgttcgacaatcacaatttcatgaaaatcatgatgatgttcaggaaaatccgcctgcgggagccggggttctatcgccacggacgcgttaccagacggaaaaaaatccacactatgtaatacggtcatactggcctcctgatgtcgtcaacacggcgaaatagtaatcacgaggtcaggttcttaccttaaattttcgacggaaaaccacgtaaaaaacgtcgatttttcaagatacagcgtgaattttcaggaaatgcggtgagcatcacatcaccacaattcagcaaattgtgaacatcatcacgttcatctttccctggttgccaatggcccattttcctgtcagtaacgagaaggtcgcgaattcaggcgctttttagactggtcgtaatgaacatttaaatgaattcccttgggactctagagatccgcgggggcccaggaggggggatctggcatttttgggaggtgtgaaatgagtgagaagatcgtcaactcgtggaacgaatgggatgagctcgaggagatggtggtcggcattgcggactatgccagcttcgaaccgaaagagccaggcaaccatcccaaactgcgcaaccagaacctggccgaaatcatccccttcccaagcggcccaaaggacccgaaggtgctggagaaagcgaacgaagagctgaatgggctggcttacctgctgaaggaccacgatgtgatcgtgcgtcgtcccgagaagatcgacttcaccaagagcctgaaaaccccgtatttcgaggttgccaaccagtactgcggcgtttgtcctcgcgacgtgatgatcacgtttggcaacgaaatcatggaagcgaccatgtccaaacgtgcacgcttcttcgaatacctcccctatcggaagctggtctacgagtactggaacaaggacgagcacatgatctggaacgcagccccgaaaccgaccatgcaggatagcatgtacctggaaaacttctgggagctctcgctggaagaacgcttcaagcggatgcacgacttcgaattctgcatcacccaagacgaggtgatcttcgatgccgccgattgctcccgcttgggtaaggacatcctggtgcaggaaagcatgaccaccaatcgcactggcatccgctggctgaagaagcatctcgaaccacgcggctttcgcgtccatccggtgcacttcccgttggacttcttccctagccacatcgactgcacgttcgtaccgttgcgtccgggtctgatcctgaccaatccggaacgcccgattcgcgaggaagaggagaagatcttcaaggagaatggctgggagctgatcaccgtaccgcagcctacctgctcgaacgacgagatgcccatgttctgccagagctcgaaatggctgtccatgaacgtcctgagcattagtcccaccaaggtgatctgcgaagaacgggaaaagccgctgcaagaactgctggacaagcacgggttcgaagtctttcccttgcctttccgccatgtgtttgagttcggtggcagctttcactgtgccacgtgggatattcgccgcaagggcgagtgcgaggactacctgccgaacctgaactaccagccgatttgcggctgacgcggatccctcgagcacgcgagagtagggaactgccaggcatcaaataaaacgaaaggctcagtcgaaagactgggcctttcgttttatctgttgtttgtcggtgaacgctctcctgagtaggacaaatccgccgggagcggatttgaacgatgataagctgtcaaacatgagaattcttgaagacgaaagggcctcgtgtgtacaaacgttcgtcaaaagggcgacacaaaattcctgcaggggccggcccagcgccggcggtcgagtggcgacggcgcggcttgtccgcgccctggtagattgcctggccgtaggccagccatttttgagcggccagcggccgcgataggccgacgcgaagcggcggggcgtagggagcgcagcgaccgaagggtaggcgctttttgcagctcttcggctgtgcgctggccagacagttatgcacaggccaggcgggttttaagagttttaataagttttaaagagttttaggcggaaaaatcgccttttttctcttttatatcagtcacttacatgtgtgaccggttcccaatgtacggctttgggttcccaatgtacgggttccggttcccaatgtacggctttgggttcccaatgtacgtgctatccacaggaaagagaccttttcgacctttttcccctgctagggcaatttgccctagcatctgctccgtacattaggaaccggcggatgcttcgccctcgatcaggttgcggtagcgcatgactaggatcgggccagcctgccccgcctcctccttcaaatcgtactccggcaggtcatttgacccgatcagcttgcgcacggtgaaacagaacttcttgaactctccggcgctgccactgcgttcgtagatcgtcttgaacaaccatctggcttctgccttgcctgcggcgcggcgtgccaggcggtagagaaaacggccgatgccgggatcgatcaaaaagtaatcggggtgaaccgtcagcacgtccgggttcttgccttctgtgatctcgcggtacatccaatcaactagctcgatctcgatgtactccggccgcccggtttcgctctttacgatcttgtagcggctaatcaaggcttcaccctcggataccgtcaccaggcggccgttcttggccttcttcgtacgctgcatggcaacgtgcgtggtgtttaaccgaatgcaggtttctaccaggtcgtctttctgctttccgccatcggctcgccggcagaacttgagtacgtccgcaacgtgtggacggaacacgcggccgggcttgtctcccttcccttcccggtatcggttcatggattcggttagatgggaaaccgccatcagtaccaggtcgtaatcccacacactggccatgccggccggccctgcggaaacctctacgtgcccgtctggaagctcgtagcggatcacctcgccagctcgtcggtcacgcttcgacagacggaaaacggccacgtccatgatgctgcgactatcgcgggtgcccacgtcatagagcatcggaacgaaaaaatctggttgctcgtcgcccttgggcggcttcctaatcgacggcgcaccggctgccggcggttgccgggattctttgcggattcgatcagcggccgcttgccacgattcaccggggcgtgcttctgcctcgatgcgttgccgctgggcggcctgcgcggccttcaacttctccaccaggtcatcacccagcgccgcgccgatttgtaccgggccggatggtttgcgaccgctcacgccgattcctcgggcttgggggttccagtgccattgcagggccggcagacaacccagccgcttacgcctggccaaccgcccgttcctccacacatggggcattccacggcgtcggtgcctggttgttcttgattttccatgccgcctcctttagccgctaaaattcatctactcatttattcatttgctcatttactctggtagctgcgcgatgtattcagatagcagctcggtaatggtcttgccttggcgtaccgcgtacatcttcagcttggtgtgatcctccgccggcaactgaaagttgacccgcttcatggctggcgtgtctgccaggctggccaacgttgcagccttgctgctgcgtgcgctcggacggccggcacttagcgtgtttgtgcttttgctcattttctctttacctcattaactcaaatgagttttgatttaatttcagcggccagcgcctggacctcgcgggcagcgtcgccctcgggttctgattcaagaacggttgtgccggcggcggcagtgcctgggtagctcacgcgctgcgtgatacgggactcaagaatgggcagctcgtacccggccagcgcctcggcaacctcaccgccgatgcgcgtgcctttgatcgcccgcgacacgacaaaggccgcttgtagccttccatccgtgacctcaatgcgctgcttaaccagctccaccaggtcggcggtggcccatatgtcgtaagggcttggctgcaccggaatcagcacgaagtcggctgccttgatcgcggacacagccaagtccgccgcctggggcgctccgtcgatcactacgaagtcgcgccggccgatggccttcacgtcgcggtcaatcgtcgggcggtcgatgccgacaacggttagcggttgatcttcccgcacggccgcccaatcgcgggcactgccctggggatcggaatcgactaacagaacatcggccccggcgagttgcagggcgcgggctagatgggttgcgatggtcgtcttgcctgacccgcctttctggttaagtacagcgataaccttcatgcgttccccttgcgtatttgtttatttactcatcgcatcatatacgcagcgaccgcatgacgcaagctgttttactcaaatacacatcacctttttagacggcggcgctcggtttcttcagcggccaagctggccggccaggccgccagcttggcatcagacaaaccggccaggatttcatgcagccgcacggttccggatgagcattca

SEQ ID NO: 39 - DNA, 921 bp, Pseudomonas putida
  CDS (1)..(921)
atgagcgctaggcactttctctccctgctggacttcaccaccgacgaattgctcggggtgatccgccacggcatcgagctgaaggacctgcgcaagcgaggcgtgctgttcgaaccgctgaagaaccgtgtgctaggcatgatcttcgaaaagtcctcgacccgtacccgtgtgtcgttcgaggccggcatgatccagctcggcggccaggccatcttcctgtcgccccgcgacacccagctgggccgcggcgagccaattggtgacagcgccatcgtgctgtcgagcatggttgatgtggtgatgatccggacccacgcccacagcaccctgaccgagttcgccgccaagtcgcgtgtgcccgtgatcaacggcctgtccgacgaatcgcacccgtgccaactgctggccgacatgcagaccttcgttgaacaccgcggctcgattcagggcaagaccgtgacctggatcggcgatggcttcaacatgtgcaactcctatatcgaagccgccaggcagttcgatttccagctgcgcatcgcctgccccgaaggctatgagccggatcaacgcttcatggcactgggcggcgaccgcgtgcagatcatccgggatgccagggaagctgtgcgtgatgcacacctggtggtcaccgatgtctggacttccatgggtcaggaggaggaaactgcacggcgcctggcgcatttcgcgccttaccaggtcacccgcgaactgctcgacctggctgcacccgatgtcctcttcatgcactgcctgcccgcccaccgtggcgaggaaatcagccaggacctgctcgacgacccacgttcggtcgcctgggacgaggctgaaaaccgcctgcatgcacagaaggcgcttctcgaattccttgtagaaccggcttaccaccacgcatga

SEQ ID NO: 40 - protein, 306 aa, Pseudomonas putida
MSARHFLSLLDFTTDELLGVIRHGIELKDLRKRGVLFEPLKNRVLGMIFEKSSTRTRVSFEAGMIQLGGQAIFLSPRDTQLGRGEPIGDSAIVLSSMVDVVMIRTHAHSTLTEFAAKSRVPVINGLSDESHPCQLLADMQTFVEHRGSIQGKTVTWIGDGFNMCNSYIEAARQFDFQLRIACPEGYEPDQRFMALGGDRVQIIRDAREAVRDAHLVVTDVWTSMGQEEETARRLAHFAPYQVTRELLDLAAPDVLFMHCLPAHRGEEISQDLLDDPRSVAWDEAENRLHAQKALLEFLVEPAYHHA

SEQ ID NO: 41 - DNA, 1218 bp, Pseudomonas putida
  CDS (1)..(1218)
atggcggacgtaaaaaaggtcgtactggcgtattccggcggccttgatacttcggtgattctcaagtggctgcaggatacctacaactgcgaagtggtgaccttcaccgctgacctggggcagggcgaagaggtcgaaccggcccgtgccaaggcccaggcaatgggcgttaaagagatctacatcgacgacctgcgcgaagaattcgtgcgtgatttcgtgttcccgatgttccgcgccaacaccgtctacgaaggcgagtacctgctgggtacttccatcgcccgtccgctgatcgccaagcgcctgatcgaaatcgccaacgaaaccggcgctgacgccatttcccatggcgccaccggcaagggtaacgaccaggtgcgcttcgagctgggtgcctatgccctgaagccaggcgtcaaggtcatcgctccatggcgcgagtgggacctgctgtcccgcgaaaagctgatggactacgccgagaagcacggcatcccgatcgagcgccacggcaagaagaagtcgccgtactcgatggacgccaacctgctgcacatctcctacgagggcggtgtcctggaagatacctggaccgagcacgaagaagacatgtggcgctggagtgtctcgcctgagaatgccccggaccaggctacctacatcgagctgacctaccgcaatggtgacatcgttgccatcgacggcgtcgagaaatccccggccaccgtcctggcagacctgaaccgtatcggtggtgccaacggcatcggccgtctggacatcgtcgaaaaccgttacgtcggcatgaagtcgcgcggttgctacgaaacgcctggcggtaccatcatgctcaaggcacaccgtgccatcgagtcgatcaccctggaccgcgaagtcgctcacctgaaagatgagctgatgccaaagtatgccagcctgatctacaccggctactggtggagcccggagcgtctgatgctgcaacagatgatcgatgcttcgcaggtcaacgtgaatggtgtggtgcgcctgaaactgtacaagggcaacgtgaccgtggttggccgcaagtcggacgattcgctgttcgatgccaacatcgccacctttgaagaagatggtggtgcctacaaccaggcagatgctgctggcttcatcaagctcaatgcactgcgtatgcgcattgccgccaacaagggccgttcgctgctctga

SEQ ID NO: 42 - protein, 405 aa, Pseudomonas putida
MADVKKVVLAYSGGLDTSVILKWLQDTYNCEVVTFTADLGQGEEVEPARAKAQAMGVKEIYIDDLREEFVRDFVFPMFRANTVYEGEYLLGTSIARPLIAKRLIEIANETGADAISHGATGKGNDQVRFELGAYALKPGVKVIAPWREWDLLSREKLMDYAEKHGIPIERHGKKKSPYSMDANLLHISYEGGVLEDTWTEHEEDMWRWSVSPENAPDQATYIELTYRNGDIVAIDGVEKSPATVLADLNRIGGANGIGRLDIVENRYVGMKSRGCYETPGGTIMLKAHRAIESITLDREVAHLKDELMPKYASLIYTGYWWSPERLMLQQMIDASQVNVNGVVRLKLYKGNVTVVGRKSDDSLFDANIATFEEDGGAYNQADAAGFIKLNALRMRIAANKGRSLL

SEQ ID NO: 43 - DNA, 1407 bp, Pseudomonas putida
  CDS (1)..(1407)
atgagtgaatccatgagcaccgagaagaccaatcagtcctggggcggccgcttcagtgagcccgtcgacgccttcgtcgcccgtttcaccgcctcggtagatttcgacaagcgcctgtaccgtcacgacatcatgggttcgattgcccatgccaccatgctggcgcaggtcggcgtgctcagtgatgccgagcgcgacaccatcatcgatggcctgaaaaccatccagggcgagattgaagccggcaacttcgactggcgtgtcgacctcgaagacgtgcacatgaacatcgaagcacgcctgaccgaccgcatcggcatcaccggcaagaagctgcatactgggcgtagccgcaacgaccaggtggccaccgacatccgcctttggctgcgcgacgaaatcgacctgatcctgggcgaaatcacccgcctgcagcagggcctgctggagcaggcagagcgtgaagccgaaaccatcatgcctggtttcacccacctgcagacggcgcagccggtcacctttggccaccacctgctggcgtggttcgaaatgctcagccgcgactatgagcgcctggtcgactgccgcaagcgcaccaaccgcatgccactgggcagcgccgcgctggccggcaccacctacccgatcgaccgtgaactgacctgcaagctgctgggctttgaagccgtggccggcaactcgctggatggcgtgtcggaccgtgatttcgccatcgaattctgcgccgctgccagcgtggcgatgatgcacctttcgcgcttctccgaagagctggtgctgtggaccagcgcgcagttccagttcatcgaccttccggaccgcttctgcactggcagctcgatcatgccgcagaaaaagaacccggacgtgccagagctggtacgtggcaagagcggccgcgtgttcggcgccctgaccggcctgctgaccctgatgaaaggccaaccgctggcctacaacaaggacaaccaggaagacaaggaaccgctgttcgacgccgccgataccctgcgcgactcgctgcgggccttcgctgacatgatcccggcgatcaagcccaagcacgccatcatgcgtgaagcggccctgcgcggtttctccaccgctaccgacctggctgactatctggttcgccgtggcctgccgttccgtgactgccacgagatcgttggccacgcggtgaagtatggtgtggacactggcaaggacctggccgagatgagcctggacgaactgcgccaattcagcgaccagatcgagcaggacgtgtttgccgtgctgacgctggaaggctcggtgaatgcgcgtgaccacattggtggtacggcgccggcgcaggtgcgtgctgccgtcgttcgtggcaaggccctgttggcgtctcgctaa

SEQ ID NO: 44 - protein, 468 aa, Pseudomonas putida
MSESMSTEKTNQSWGGRFSEPVDAFVARFTASVDFDKRLYRHDIMGSIAHATMLAQVGVLSDAERDTIIDGLKTIQGEIEAGNFDWRVDLEDVHMNIEARLTDRIGITGKKLHTGRSRNDQVATDIRLWLRDEIDLILGEITRLQQGLLEQAEREAETIMPGFTHLQTAQPVTFGHHLLAWFEMLSRDYERLVDCRKRTNRMPLGSAALAGTTYPIDRELTCKLLGFEAVAGNSLDGVSDRDFAIEFCAAASVAMMHLSRFSEELVLWTSAQFQFIDLPDRFCTGSSIMPQKKNPDVPELVRGKSGRVFGALTGLLTLMKGQPLAYNKDNQEDKEPLFDAADTLRDSLRAFADMIPAIKPKHAIMREAALRGFSTATDLADYLVRRGLPFRDCHEIVGHAVKYGVDTGKDLAEMSLDELRQFSDQIEQDVFAVLTLEGSVNARDHIGGTAPAQVRAAVVRGKALLASR

SEQ ID NO: 45 - DNA, 3701 bp, Pseudomonas putida
tctagagatccgcgggggcccgacctgcataccgttgcagataaggtagtcactcatgagcgctaggcactttctctccctgctggacttcaccaccgacgaattgctcggggtgatccgccacggcatcgagctgaaggacctgcgcaagcgaggcgtgctgttcgaaccgctgaagaaccgtgtgctaggcatgatcttcgaaaagtcctcgacccgtacccgtgtgtcgttcgaggccggcatgatccagctcggcggccaggccatcttcctgtcgccccgcgacacccagctgggccgcggcgagccaattggtgacagcgccatcgtgctgtcgagcatggttgatgtggtgatgatccggacccacgcccacagcaccctgaccgagttcgccgccaagtcgcgtgtgcccgtgatcaacggcctgtccgacgaatcgcacccgtgccaactgctggccgacatgcagaccttcgttgaacaccgcggctcgattcagggcaagaccgtgacctggatcggcgatggcttcaacatgtgcaactcctatatcgaagccgccaggcagttcgatttccagctgcgcatcgcctgccccgaaggctatgagccggatcaacgcttcatggcactgggcggcgaccgcgtgcagatcatccgggatgccagggaagctgtgcgtgatgcacacctggtggtcaccgatgtctggacttccatgggtcaggaggaggaaactgcacggcgcctggcgcatttcgcgccttaccaggtcacccgcgaactgctcgacctggctgcacccgatgtcctcttcatgcactgcctgcccgcccaccgtggcgaggaaatcagccaggacctgctcgacgacccacgttcggtcgcctgggacgaggctgaaaaccgcctgcatgcacagaaggcgcttctcgaattccttgtagaaccggcttaccaccacgcatgagtcaaccgtacaaccccgtggagtgatggcatggcggacgtaaaaaaggtcgtactggcgtattccggcggccttgatacttcggtgattctcaagtggctgcaggatacctacaactgcgaagtggtgaccttcaccgctgacctggggcagggcgaagaggtcgaaccggcccgtgccaaggcccaggcaatgggcgttaaagagatctacatcgacgacctgcgcgaagaattcgtgcgtgatttcgtgttcccgatgttccgcgccaacaccgtctacgaaggcgagtacctgctgggtacttccatcgcccgtccgctgatcgccaagcgcctgatcgaaatcgccaacgaaaccggcgctgacgccatttcccatggcgccaccggcaagggtaacgaccaggtgcgcttcgagctgggtgcctatgccctgaagccaggcgtcaaggtcatcgctccatggcgcgagtgggacctgctgtcccgcgaaaagctgatggactacgccgagaagcacggcatcccgatcgagcgccacggcaagaagaagtcgccgtactcgatggacgccaacctgctgcacatctcctacgagggcggtgtcctggaagatacctggaccgagcacgaagaagacatgtggcgctggagtgtctcgcctgagaatgccccggaccaggctacctacatcgagctgacctaccgcaatggtgacatcgttgccatcgacggcgtcgagaaatccccggccaccgtcctggcagacctgaaccgtatcggtggtgccaacggcatcggccgtctggacatcgtcgaaaaccgttacgtcggcatgaagtcgcgcggttgctacgaaacgcctggcggtaccatcatgctcaaggcacaccgtgccatcgagtcgatcaccctggaccgcgaagtcgctcacctgaaagatgagctgatgccaaagtatgccagcctgatctacaccggctactggtggagcccggagcgtctgatgctgcaacagatgatcgatgcttcgcaggtcaacgtgaatggtgtggtgcgcctgaaactgtacaagggcaacgtgaccgtggttggccgcaagtcggacgattcgctgttcgatgccaacatcgccacctttgaagaagatggtggtgcctacaaccaggcagatgctgctggcttcatcaagctcaatgcactgcgtatgcgcattgccgccaacaagggccgttcgctgctctgattgctatcgacgccactttttcgttcacgcctgcaatgagtgaatccatgagcaccgagaagaccaatcagtcctggggcggccgcttcagtgagcccgtcgacgccttcgtcgcccgtttcaccgcctcggtagatttcgacaagcgcctgtaccgtcacgacatcatgggttcgattgcccatgccaccatgctggcgcaggtcggcgtgctcagtgatgccgagcgcgacaccatcatcgatggcctgaaaaccatccagggcgagattgaagccggcaacttcgactggcgtgtcgacctcgaagacgtgcacatgaacatcgaagcacgcctgaccgaccgcatcggcatcaccggcaagaagctgcatactgggcgtagccgcaacgaccaggtggccaccgacatccgcctttggctgcgcgacgaaatcgacctgatcctgggcgaaatcacccgcctgcagcagggcctgctggagcaggcagagcgtgaagccgaaaccatcatgcctggtttcacccacctgcagacggcgcagccggtcacctttggccaccacctgctggcgtggttcgaaatgctcagccgcgactatgagcgcctggtcgactgccgcaagcgcaccaaccgcatgccactgggcagcgccgcgctggccggcaccacctacccgatcgaccgtgaactgacctgcaagctgctgggctttgaagccgtggccggcaactcgctggatggcgtgtcggaccgtgatttcgccatcgaattctgcgccgctgccagcgtggcgatgatgcacctttcgcgcttctccgaagagctggtgctgtggaccagcgcgcagttccagttcatcgaccttccggaccgcttctgcactggcagctcgatcatgccgcagaaaaagaacccggacgtgccagagctggtacgtggcaagagcggccgcgtgttcggcgccctgaccggcctgctgaccctgatgaaaggccaaccgctggcctacaacaaggacaaccaggaagacaaggaaccgctgttcgacgccgccgataccctgcgcgactcgctgcgggccttcgctgacatgatcccggcgatcaagcccaagcacgccatcatgcgtgaagcggccctgcgcggtttctccaccgctaccgacctggctgactatctggttcgccgtggcctgccgttccgtgactgccacgagatcgttggccacgcggtgaagtatggtgtggacactggcaaggacctggccgagatgagcctggacgaactgcgccaattcagcgaccagatcgagcaggacgtgtttgccgtgctgacgctggaaggctcggtgaatgcgcgtgaccacattggtggtacggcgccggcgcaggtgcgtgctgccgtcgttcgtggcaaggccctgttggcgtctcgctaatcccccaaggctcgagcacgcgagagtagggaact

SEQ ID NO: 46 - DNA, 23 bp, synthetic oligonucleotide
ggatccgcgtcagccgcaaatcg

SEQ ID NO: 47 - DNA, 45 bp, synthetic oligonucleotide
tttgcggctgacgcggatcccgacctgcataccgttgcagataag

SEQ ID NO: 48 - DNA, 22 bp, synthetic oligonucleotide
agttccctactctcgcgtgctc

SEQ ID NO: 49 - DNA, 13891 bp, various
tcaggcgggcaagaatgtgaataaaggccggataaaacttgtgcttatttttctttacggtctttaaaaaggccgtaatatccagctgaacggtctggttataggtacattgagcaactgactgaaatgcctcaaaatgttctttacgatgccattgggatatatcaacggtggtatatccagtgatttttttctccattttagcttccttagctcctgaaaatctcgataactcaaaaaatacgcccggtagtgatcttatttcattatggtgaaagttggaacctcttacgtgccgatcaacgtctcattttcgccaaaagttggcccagggcttcccggtatcaacagggacaccaggatttatttattctgcgaagtgatcttccgtcacaggtatttattcggcgcaaagtgcgtcgggtgatgctgccaacttactgatttagtgtatgatggtgtttttgaggtgctccagtggcttctgtttctatcagctgtccctcctgttcagctactgacggggtggtgcgtaacggcaaaagcaccgccggacatcagcgctagcggagtgtatactggcttactatgttggcactgatgagggtgtcagtgaagtgcttcatgtggcaggagaaaaaaggctgcaccggtgcgtcagcagaatatgtgatacaggatatattccgcttcctcgctcactgactcgctacgctcggtcgttcgactgcggcgagcggaaatggcttacgaacggggcggagatttcctggaagatgccaggaagatacttaacagggaagtgagagggccgcggcaaagccgtttttccataggctccgcccccctgacaagcatcacgaaatctgacgctcaaatcagtggtggcgaaacccgacaggactataaagataccaggcgtttccccctggcggctccctcgtgcgctctcctgttcctgcctttcggtttaccggtgtcattccgctgttatggccgcgtttgtctcattccacgcctgacactcagttccgggtaggcagttcgctccaagctggactgtatgcacgaaccccccgttcagtccgaccgctgcgccttatccggtaactatcgtcttgagtccaacccggaaagacatgcaaaagcaccactggcagcagccactggtaattgatttagaggagttagtcttgaagtcatgcgccggttaaggctaaactgaaaggacaagttttggtgactgcgctcctccaagccagttacctcggttcaaagagttggtagctcagagaaccttcgaaaaaccgccctgcaaggcggttttttcgttttcagagcaagagattacgcgcagaccaaaacgatctcaagaagatcatcttattaatcagataaaatatttctagatttcagtgcaatttatctcttcaaatgtagcacctgaagtcagccccatacgatataagttgtaattctcatgtttgacagcttatcatcgataagctttaatgcggtagtttatcacagttaaattgctaacgcagtcaggcaccgtgtatgaaatctaacaatgcgctcatcgtcatcctcggcaccgtcaccctggatgctgtaggcataggcttggttatgccggtactgccgggcctcttgcgggatatcgtccattccgacagcatcgccagtcactatggcgtgctgctagcgctatatgcgttgatgcaatttctatgcgcacccgttctcggagcactgtccgaccgctttggccgccgcccagtcctgctcgcttcgctacttggagccactatcgactacgcgatcatggcgaccacacccgtcctgtggatcctctacgccggacgcatcgtggccggcatcaccggcgccacaggtgcggttgctggcgcctatatcgccgacatcaccgatggggaagatcgggctcgccacttcgggctcatgagcgcttgtttcggcgtgggtatggtggcaggccccgtggccgggggactgttgggcgccatctccttgcatgcaccattccttgcggcggcggtgctcaacggcctcaacctactactgggctgcttcctaatgcaggagtcgcataagggagagcgtcgaccgatgcccttgagagccttcaacccagtcagctccttccggtgggcgcggggcatgactatcgtcgccgcacttatgactgtcttctttatcatgcaactcgtaggacaggtgccggcagcgctctgggtcattttcggcgaggaccgctttcgctggagcgcgacgatgatcggcctgtcgcttgcggtattcggaatcttgcacgccctcgctcaagccttcgtcactggtcccgccaccaaacgtttcggcgagaagcaggccattatcgccggcatggcggccgacgcgctgggctacgtcttgctggcgttcgcgacgcgaggctggatggccttccccattatgattcttctcgcttccggcggcatcgggatgcccgcgttgcaggccatgctgtccaggcaggtagatgacgaccatcagggacagcttcaaggatcgctcgcggctcttaccagcctaacttcgatcattggaccgctgatcgtcacggcgatttatgccgcctcggcgagcacatggaacgggttggcatggattgtaggcgccgccctataccttgtctgcctccccgcgttgcgtcgcggtgcatggagccgggccacctcgacctgaatggaagccggcggcacctcgctaacggattcaccactccaagaattggagccaatcaattcttgcggagaactgtgaatgcgcaaaccaacccttggcagaacatatccatcgcgtccgccatctccagcagccgcacgcggcgcatctcgggcagcgttgggtcctggccacgggtgcgcatgatcgtgctcctgtcgttgaggacccggctaggctggcggggttgccttactggttagcagaatgaatcaccgatacgcgagcgaacgtgaagcgactgctgctgcaaaacgtctgcgacctgagcaacaacatgaatggtcttcggtttccgtgtttcgtaaagtctggaaacgcggaagtcccctacgtgctgctgaagttgcccgcaacagagagtggaaccaaccggtgataccacgatactatgactgagagtcaacgccatgagcggcctcatttcttattctgagttacaacagtccgcaccgctgtccggtagctccttccggtgggcgcggggcatgactatcgtcgccgcacttatgactgtcttctttatcatgcaactcgtaggacaggtgccggcagcgcccaacagtcccccggccacggggcctgccaccatacccacgccgaaacaagcgccctgcaccattatgttccggatctgcatcgcaggatgctgctggctaccctgtggaacacctacatctgtattaacgaagcgctaaccgtttttatcaggctctgggaggcagaataaatgatcatatcgtcaattattacctccacggggagagcctgagcaaactggcctcaggcatttgagaagcacacggtcacactgcttccggtagtcaataaaccggtaaaccagcaatagacataagcggctatttaacgaccctgccctgaaccgacgaccgggtcgaatttgctttcgaatttctgccattcatccgcttattatcacttattcaggcgtagcaccaggcgtttaagggcaccaataactgccttaaaaaaattacgccccgccctgccactcatcgcagtactgttgtaattcattaagcattctgccgacatggaagccatcacaaacggcatgatgaacctgaatcgccagcggcatcagcaccttgtcgccttgcgtataatatttgcccatggatttaaatttaatctttctgcgaattgagatgacgccactggctgggcgtcatcccggtttcccgggtaaacaccaccgaaaaatagttactatcttcaaagccacattcggtcgaaatatcactgattaacaggcggctatgctggagaagatattgcgcatgacacactctgacctgtcgcagatattgattgatggtcattccagtctgctggcgaaattgctgacgcaaaacgcgctcactgcacgatgcctcatcacaaaatttatccagcgcaaagggacttttcaggctagccgccagccgggtaatcagcttatccagcaacgtttcgctggatgttggcggcaacgaatcactggtgtaacgatggcgattcagcaacatcaccaactgcccgaacagcaactcagccatttcgttagcaaacggcacatgctgactactttcatgctcaagctgaccgataacctgccgcgcctgcgccatccccatgctacctaagcgccagtgtggttgccctgcgctggcgttaaatcccggaatcgccccctgccagtcaagattcagcttcagacgctccgggcaataaataatattctgcaaaaccagatcgttaacggaagcgtaggagtgtttatcgtcagcatgaatgtaaaagagatcgccacgggtaatgcgataagggcgatcgttgagtacatgcaggccattaccgcgccagacaatcaccagctcacaaaaatcatgtgtatgttcagcaaagacatcttgcggataacggtcagccacagcgactgcctgctggtcgctggcaaaaaaatcatctttgagaagttttaactgatgcgccaccgtggctacctcggccagagaacgaagttgattattcgcaatatggcgtacaaatacgttgagaagattcgcgttattgcagaaagccatcccgtccctggcgaatatcacgcggtgaccagttaaactctcggcgaaaaagcgtcgaaaagtggttactgtcgctgaatccacagcgataggcgatgtcagtaacgctggcctcgctgtggcgtagcagatgtcgggctttcatcagtcgcaggcggttcaggtatcgctgaggcgtcagtcccgtttgctgcttaagctgccgatgtagcgtacgcagtgaaagagaaaattgatccgccacggcatcccaattcacctcatcggcaaaatggtcctccagccaggccagaagcaagttgagacgtgatgcgctgttttccaggttctcctgcaaactgcttttacgcagcaagagcagtaattgcataaacaagatctcgcgactggcggtcgagggtaaatcattttccccttcctgctgttccatctgtgcaaccagctgtcgcacctgctgcaatacgctgtggttaacgcgccagtgagacggatactgcccatccagctcttgtggcagcaactgattcagcccggcgagaaactgaaatcgatccggcgagcgatacagcacattggtcagacacagattatcggtatgttcatacagatgccgatcatgatcgcgtacgaaacagaccgtgccaccggtgatggtatagggctgcccattaaacacatgaatacccgtgccatgttcgacaatcacaatttcatgaaaatcatgatgatgttcaggaaaatccgcctgcgggagccggggttctatcgccacggacgcgttaccagacggaaaaaaatccacactatgtaatacggtcatactggcctcctgatgtcgtcaacacggcgaaatagtaatcacgaggtcaggttcttaccttaaattttcgacggaaaaccacgtaaaaaacgtcgatttttcaagatacagcgtgaattttcaggaaatgcggtgagcatcacatcaccacaattcagcaaattgtgaacatcatcacgttcatctttccctggttgccaatggcccattttcctgtcagtaacgagaaggtcgcgaattcaggcgctttttagactggtcgtaatgaacatttaaatgaattcccttgggactctagagatccgcgggggcccaggaggggggatctggcatttttgggaggtgtgaaatgagtgagaagatcgtcaactcgtggaacgaatgggatgagctcgaggagatggtggtcggcattgcggactatgccagcttcgaaccgaaagagccaggcaaccatcccaaactgcgcaaccagaacctggccgaaatcatccccttcccaagcggcccaaaggacccgaaggtgctggagaaagcgaacgaagagctgaatgggctggcttacctgctgaaggaccacgatgtgatcgtgcgtcgtcccgagaagatcgacttcaccaagagcctgaaaaccccgtatttcgaggttgccaaccagtactgcggcgtttgtcctcgcgacgtgatgatcacgtttggcaacgaaatcatggaagcgaccatgtccaaacgtgcacgcttcttcgaatacctcccctatcggaagctggtctacgagtactggaacaaggacgagcacatgatctggaacgcagccccgaaaccgaccatgcaggatagcatgtacctggaaaacttctgggagctctcgctggaagaacgcttcaagcggatgcacgacttcgaattctgcatcacccaagacgaggtgatcttcgatgccgccgattgctcccgcttgggtaaggacatcctggtgcaggaaagcatgaccaccaatcgcactggcatccgctggctgaagaagcatctcgaaccacgcggctttcgcgtccatccggtgcacttcccgttggacttcttccctagccacatcgactgcacgttcgtaccgttgcgtccgggtctgatcctgaccaatccggaacgcccgattcgcgaggaagaggagaagatcttcaaggagaatggctgggagctgatcaccgtaccgcagcctacctgctcgaacgacgagatgcccatgttctgccagagctcgaaatggctgtccatgaacgtcctgagcattagtcccaccaaggtgatctgcgaagaacgggaaaagccgctgcaagaactgctggacaagcacgggttcgaagtctttcccttgcctttccgccatgtgtttgagttcggtggcagctttcactgtgccacgtgggatattcgccgcaagggcgagtgcgaggactacctgccgaacctgaactaccagccgatttgcggctgacgcggatcccgacctgcataccgttgcagataaggtagtcactcatgagcgctaggcactttctctccctgctggacttcaccaccgacgaattgctcggggtgatccgccacggcatcgagctgaaggacctgcgcaagcgaggcgtgctgttcgaaccgctgaagaaccgtgtgctaggcatgatcttcgaaaagtcctcgacccgtacccgtgtgtcgttcgaggccggcatgatccagctcggcggccaggccatcttcctgtcgccccgcgacacccagctgggccgcggcgagccaattggtgacagcgccatcgtgctgtcgagcatggttgatgtggtgatgatccggacccacgcccacagcaccctgaccgagttcgccgccaagtcgcgtgtgcccgtgatcaacggcctgtccgacgaatcgcacccgtgccaactgctggccgacatgcagaccttcgttgaacaccgcggctcgattcagggcaagaccgtgacctggatcggcgatggcttcaacatgtgcaactcctatatcgaagccgccaggcagttcgatttccagctgcgcatcgcctgccccgaaggctatgagccggatcaacgcttcatggcactgggcggcgaccgcgtgcagatcatccgggatgccagggaagctgtgcgtgatgcacacctggtggtcaccgatgtctggacttccatgggtcaggaggaggaaactgcacggcgcctggcgcatttcgcgccttaccaggtcacccgcgaactgctcgacctggctgcacccgatgtcctcttcatgcactgcctgcccgcccaccgtggcgaggaaatcagccaggacctgctcgacgacccacgttcggtcgcctgggacgaggctgaaaaccgcctgcatgcacagaaggcgcttctcgaattccttgtagaaccggcttaccaccacgcatgagtcaaccgtacaaccccgtggagtgatggcatggcggacgtaaaaaaggtcgtactggcgtattccggcggccttgatacttcggtgattctcaagtggctgcaggatacctacaactgcgaagtggtgaccttcaccgctgacctggggcagggcgaagaggtcgaaccggcccgtgccaaggcccaggcaatgggcgttaaagagatctacatcgacgacctgcgcgaagaattcgtgcgtgatttcgtgttcccgatgttccgcgccaacaccgtctacgaaggcgagtacctgctgggtacttccatcgcccgtccgctgatcgccaagcgcctgatcgaaatcgccaacgaaaccggcgctgacgccatttcccatggcgccaccggcaagggtaacgaccaggtgcgcttcgagctgggtgcctatgccctgaagccaggcgtcaaggtcatcgctccatggcgcgagtgggacctgctgtcccgcgaaaagctgatggactacgccgagaagcacggcatcccgatcgagcgccacggcaagaagaagtcgccgtactcgatggacgccaacctgctgcacatctcctacgagggcggtgtcctggaagatacctggaccgagcacgaagaagacatgtggcgctggagtgtctcgcctgagaatgccccggaccaggctacctacatcgagctgacctaccgcaatggtgacatcgttgccatcgacggcgtcgagaaatccccggccaccgtcctggcagacctgaaccgtatcggtggtgccaacggcatcggccgtctggacatcgtcgaaaaccgttacgtcggcatgaagtcgcgcggttgctacgaaacgcctggcggtaccatcatgctcaaggcacaccgtgccatcgagtcgatcaccctggaccgcgaagtcgctcacctgaaagatgagctgatgccaaagtatgccagcctgatctacaccggctactggtggagcccggagcgtctgatgctgcaacagatgatcgatgcttcgcaggtcaacgtgaatggtgtggtgcgcctgaaactgtacaagggcaacgtgaccgtggttggccgcaagtcggacgattcgctgttcgatgccaacatcgccacctttgaagaagatggtggtgcctacaaccaggcagatgctgctggcttcatcaagctcaatgcactgcgtatgcgcattgccgccaacaagggccgttcgctgctctgattgctatcgacgccactttttcgttcacgcctgcaatgagtgaatccatgagcaccgagaagaccaatcagtcctggggcggccgcttcagtgagcccgtcgacgccttcgtcgcccgtttcaccgcctcggtagatttcgacaagcgcctgtaccgtcacgacatcatgggttcgattgcccatgccaccatgctggcgcaggtcggcgtgctcagtgatgccgagcgcgacaccatcatcgatggcctgaaaaccatccagggcgagattgaagccggcaacttcgactggcgtgtcgacctcgaagacgtgcacatgaacatcgaagcacgcctgaccgaccgcatcggcatcaccggcaagaagctgcatactgggcgtagccgcaacgaccaggtggccaccgacatccgcctttggctgcgcgacgaaatcgacctgatcctgggcgaaatcacccgcctgcagcagggcctgctggagcaggcagagcgtgaagccgaaaccatcatgcctggtttcacccacctgcagacggcgcagccggtcacctttggccaccacctgctggcgtggttcgaaatgctcagccgcgactatgagcgcctggtcgactgccgcaagcgcaccaaccgcatgccactgggcagcgccgcgctggccggcaccacctacccgatcgaccgtgaactgacctgcaagctgctgggctttgaagccgtggccggcaactcgctggatggcgtgtcggaccgtgatttcgccatcgaattctgcgccgctgccagcgtggcgatgatgcacctttcgcgcttctccgaagagctggtgctgtggaccagcgcgcagttccagttcatcgaccttccggaccgcttctgcactggcagctcgatcatgccgcagaaaaagaacccggacgtgccagagctggtacgtggcaagagcggccgcgtgttcggcgccctgaccggcctgctgaccctgatgaaaggccaaccgctggcctacaacaaggacaaccaggaagacaaggaaccgctgttcgacgccgccgataccctgcgcgactcgctgcgggccttcgctgacatgatcccggcgatcaagcccaagcacgccatcatgcgtgaagcggccctgcgcggtttctccaccgctaccgacctggctgactatctggttcgccgtggcctgccgttccgtgactgccacgagatcgttggccacgcggtgaagtatggtgtggacactggcaaggacctggccgagatgagcctggacgaactgcgccaattcagcgaccagatcgagcaggacgtgtttgccgtgctgacgctggaaggctcggtgaatgcgcgtgaccacattggtggtacggcgccggcgcaggtgcgtgctgccgtcgttcgtggcaaggccctgttggcgtctcgctaatcccccaaggctcgagcacgcgagagtagggaactgccaggcatcaaataaaacgaaaggctcagtcgaaagactgggcctttcgttttatctgttgtttgtcggtgaacgctctcctgagtaggacaaatccgccgggagcggatttgaacgatgataagctgtcaaacatgagaattcttgaagacgaaagggcctcgtgtgtacaaacgttcgtcaaaagggcgacacaaaattcctgcaggggccggcccagcgccggcggtcgagtggcgacggcgcggcttgtccgcgccctggtagattgcctggccgtaggccagccatttttgagcggccagcggccgcgataggccgacgcgaagcggcggggcgtagggagcgcagcgaccgaagggtaggcgctttttgcagctcttcggctgtgcgctggccagacagttatgcacaggccaggcgggttttaagagttttaataagttttaaagagttttaggcggaaaaatcgccttttttctcttttatatcagtcacttacatgtgtgaccggttcccaatgtacggctttgggttcccaatgtacgggttccggttcccaatgtacggctttgggttcccaatgtacgtgctatccacaggaaagagaccttttcgacctttttcccctgctagggcaatttgccctagcatctgctccgtacattaggaaccggcggatgcttcgccctcgatcaggttgcggtagcgcatgactaggatcgggccagcctgccccgcctcctccttcaaatcgtactccggcaggtcatttgacccgatcagcttgcgcacggtgaaacagaacttcttgaactctccggcgctgccactgcgttcgtagatcgtcttgaacaaccatctggcttctgccttgcctgcggcgcggcgtgccaggcggtagagaaaacggccgatgccgggatcgatcaaaaagtaatcggggtgaaccgtcagcacgtccgggttcttgccttctgtgatctcgcggtacatccaatcaactagctcgatctcgatgtactccggccgcccggtttcgctctttacgatcttgtagcggctaatcaaggcttcaccctcggataccgtcaccaggcggccgttcttggccttcttcgtacgctgcatggcaacgtgcgtggtgtttaaccgaatgcaggtttctaccaggtcgtctttctgctttccgccatcggctcgccggcagaacttgagtacgtccgcaacgtgtggacggaacacgcggccgggcttgtctcccttcccttcccggtatcggttcatggattcggttagatgggaaaccgccatcagtaccaggtcgtaatcccacacactggccatgccggccggccctgcggaaacctctacgtgcccgtctggaagctcgtagcggatcacctcgccagctcgtcggtcacgcttcgacagacggaaaacggccacgtccatgatgctgcgactatcgcgggtgcccacgtcatagagcatcggaacgaaaaaatctggttgctcgtcgcccttgggcggcttcctaatcgacggcgcaccggctgccggcggttgccgggattctttgcggattcgatcagcggccgcttgccacgattcaccggggcgtgcttctgcctcgatgcgttgccgctgggcggcctgcgcggccttcaacttctccaccaggtcatcacccagcgccgcgccgatttgtaccgggccggatggtttgcgaccgctcacgccgattcctcgggcttgggggttccagtgccattgcagggccggcagacaacccagccgcttacgcctggccaaccgcccgttcctccacacatggggcattccacggcgtcggtgcctggttgttcttgattttccatgccgcctcctttagccgctaaaattcatctactcatttattcatttgctcatttactctggtagctgcgcgatgtattcagatagcagctcggtaatggtcttgccttggcgtaccgcgtacatcttcagcttggtgtgatcctccgccggcaactgaaagttgacccgcttcatggctggcgtgtctgccaggctggccaacgttgcagccttgctgctgcgtgcgctcggacggccggcacttagcgtgtttgtgcttttgctcattttctctttacctcattaactcaaatgagttttgatttaatttcagcggccagcgcctggacctcgcgggcagcgtcgccctcgggttctgattcaagaacggttgtgccggcggcggcagtgcctgggtagctcacgcgctgcgtgatacgggactcaagaatgggcagctcgtacccggccagcgcctcggcaacctcaccgccgatgcgcgtgcctttgatcgcccgcgacacgacaaaggccgcttgtagccttccatccgtgacctcaatgcgctgcttaaccagctccaccaggtcggcggtggcccatatgtcgtaagggcttggctgcaccggaatcagcacgaagtcggctgccttgatcgcggacacagccaagtccgccgcctggggcgctccgtcgatcactacgaagtcgcgccggccgatggccttcacgtcgcggtcaatcgtcgggcggtcgatgccgacaacggttagcggttgatcttcccgcacggccgcccaatcgcgggcactgccctggggatcggaatcgactaacagaacatcggccccggcgagttgcagggcgcgggctagatgggttgcgatggtcgtcttgcctgacccgcctttctggttaagtacagcgataaccttcatgcgttccccttgcgtatttgtttatttactcatcgcatcatatacgcagcgaccgcatgacgcaagctgttttactcaaatacacatcacctttttagacggcggcgctcggtttcttcagcggccaagctggccggccaggccgccagcttggcatcagacaaaccggccaggatttcatgcagccgcacggttccggatgagcattca

SEQ ID NO: 50 - DNA, 1137 bp, Pseudomonas putida
  CDS (1)..(1137)
ttgacaaagccagccatactcgcccttgccgacggcagtattttccgcggtgaagccatcggtgccgacggtcagaccgttggtgaggtggtattcaacaccgctatgaccggctaccaggaaatccttacagacccttcctacgcgcagcaaatcgttaccctgacctacccgcacatcggcaacaccggtactaccccggaagacgccgagtcgagccgcgtctggtccgctggcctggtcatccgtgacctgccgctgctggccagcaactggcgtaacacccagtcgctgcctgagtacctcaaggccaacaacgtcgtcgccatcgccggcatcgacacccgtcgcctgacccgtatcctgcgtgaaaagggcgcccagaacggctgcattctggcgggtgacaacatcagcgaagaagctgccatcgctgctgcccgcggcttcccgggcctgaagggcatggacctggccaaggtcgtctccaccaaggaacgttacgagtggcgctccagcgtgtgggagctgaaaaccgacagccacccgaccatcgacgctgccgacctgccgtaccacgtggttgccttcgactatggcgtcaagctgaacatcctgcgcatgctggtggcccgcggctgccgcgtgaccgtggtaccagcccagaccccggccagcgaagtactggcactcaacccggacggcgtgttcctgtccaacggccctggtgaccctgagccgtgcgactacgcgatccaggcgatcaaggaaatcctcgaaaccgagatcccggtattcggcatctgcctcggccaccagctgctggccctggcgtccggcgccaagaccgtgaaaatgggccacggccaccacggtgccaaccacccggtccaggacctggatactggtgtggtcatgatcaccagccagaaccacggtttcgccgttgacgaggcgaccctgccgggcaacgttcgcgccattcacaagtcgctgttcgacggcaccctgcagggtatcgagcgtaccgacaagagcgcgttcagcttccagggccaccctgaagcgagcccgggcccgaccgacgtcgcgcctctgttcgatcgtttcaccgatgccatggccaagcgccgctga

SEQ ID NO: 51 - protein, 378 aa, Pseudomonas putida
LTKPAILALADGSIFRGEAIGADGQTVGEVVFNTAMTGYQEILTDPSYAQQIVTLTYPHIGNTGTTPEDAESSRVWSAGLVIRDLPLLASNWRNTQSLPEYLKANNVVAIAGIDTRRLTRILREKGAQNGCILAGDNISEEAAIAAARGFPGLKGMDLAKVVSTKERYEWRSSVWELKTDSHPTIDAADLPYHVVAFDYGVKLNILRMLVARGCRVTVVPAQTPASEVLALNPDGVFLSNGPGDPEPCDYAIQAIKEILETEIPVFGICLGHQLLALASGAKTVKMGHGHHGANHPVQDLDTGVVMITSQNHGFAVDEATLPGNVRAIHKSLFDGTLQGIERTDKSAFSFQGHPEASPGPTDVAPLFDRFTDAMAKRR

SEQ ID NO: 52 - DNA, 3222 bp, Pseudomonas putida
  CDS (1)..(3222)
atgccaaaacgtacagacatcaaaagcatcctgattctcggcgctggcccgatcgtgatcggccaggcctgcgaattcgactactccggcgcccaggcctgtaaagccctgcgcgaggaaggtttccgcgtcatcctggtgaactccaacccagccaccatcatgaccgacccggccatggctgacgccacctacatcgagccgatcaagtggcaatcggtggccaagatcatcgagaaagagcgcccggacgccgtcctgccgaccatgggtggccagaccgccctgaactgcgccctggacctggagcgccacggcgttctggagaagttcggcgtggagatgatcggtgccaacgctgacaccatcgacaaggccgaagaccgttcgcgcttcgacaaggccatgaaggacatcggcctggagtgcccgcgctccggtatcgcccacagcatggaagaggccaatgcggtcctcgagaagctcggcttcccgtgcatcattcgcccgtcgttcaccatgggcggcaccggcggcggtatcgcttacaaccgtgaagagttcgaagaaatctgcacccgtggtctggacctgtcgccgaccaaagagctgctgatcgacgaatcgctgatcggctggaaggaatacgagatggaggtggtccgcgacaagaaggacaactgcatcatcgtctgctcgatcgagaacttcgacccgatgggtgtgcacaccggtgactcgatcactgttgccccggcacagaccctgaccgacaaggaataccagatcatgcgcaacgcctcgctggcggtgctgcgtgaaatcggtgtggaaaccggcggttccaacgtccagttcggcatttgcccgaacaccggccgcatggttgtcatcgagatgaacccgcgcgtgtcgcgttcgtccgccctggcctccaaggccaccggcttcccgatcgccaagatcgccgccaagctggccattggttacaccctcgacgagctgcagaacgacatcactggcggtcgcaccccagcgtccttcgaaccttcgatcgactacgtcgtcaccaagctgccacgcttcgccttcgagaaattcccgaaagccgacgcccgcctgaccacccagatgaaatccgtgggtgaagtcatggccatcggccgtactttccaggaatccctgcagaaagccctgcgcggcctggaagtcggcgcctgcggcctcgacccgaaagtcgacctggccagcccggaagccgccagcatcctcaagcgcgaactgaccgtgccgggtgccgagcgtatctggtacgtggctgacgccatgcgttcgggcatgacctgcgaagaaatcttcaatctgaccggcatcgacatgtggttcctggtgcagatggaagacctgatcaaggaagaagagaaggtcaagaccctggccctgtcggcaatcgacaaggactacatgctgcgcctcaagcgcaagggcttctcggaccagcgcctggcagtactgctgggtatcaccgacaagaacctgcgtcgccaccgccacaagctggaagtgttcccggtgtacaagcgcgtcgacacctgcgccgccgagttcgccaccgacaccgcctacctgtactccacctacgaggaagagtgcgaggccaacccgtcgacccgcgacaagatcatgatcctgggtggcggcccgaaccgtatcggccaaggtatcgagttcgactactgctgcgtacacgccgccctggcgctgcgtgaagacggttacgagaccatcatggtcaactgcaacccggaaaccgtctccaccgactacgacacttccgaccgcctgtacttcgagccgctgaccctggaagacgtgctggaagtctgccgcgtcgagaagccgaagggcgtgatcgttcactacggcggccagaccccgctgaagctggcccgcgctctggaagaggctggcgtgccgatcatcggtaccagccctgacgccatcgaccgcgccgaagaccgcgagcgcttccagcagatggttcagcgcctgagcctgctgcagccgccaaacgccaccgtgcgcagcgaagaagaagccatccgtgctgcgggcagcatcggctacccgctggtcgtgcgtccgtcctacgtactgggcggccgtgccatggagatcgtctacgagctggacgagctcaagcgctacctgcgtgaagcggtacaagtgtcgaacgacagcccggtactgctcgaccacttcctcaactgcgccatcgagatggacgtggatgcggtgtgcgacggcaccgacgtggtcatcggcgcgatcatgcagcacatcgagcaggccggcgtacactccggcgactcggcgtgctcgctgccaccttactcgctgagcaaggaagtgcaggacgaagtccgcgttcaggtcaagaaaatggcgctggagctgggtgtagtcggcctgatgaacgtgcagctggccctgcagggcgacaagatctacgtgatcgaagtcaacccgcgtgcctcgcgtaccgtaccgttcgtgtccaagtgcatcggcacgtccctggcgatgatcgcagcccgtgtcatggcgggtaaaaccctgaaagagctgggcttcacccaggaaatcatcccgaacttctacagcgtgaaggaagccgtcttcccgttcgccaagttcccaggggttgacccgatcctcggccctgagatgaaatcgaccggtgaagtgatgggtgtcggtgacagcttcggtgaagccttcgccaaagcccagatgggtgccagcgaagtgctgccgactggcggtaccgcgttcatcagcgtgcgcgacgacgacaagccacaagtggccggcgttgcccgcgacctgatcgccctgggcttcgaagtggttgccactgccggcaccgccaaggttatcgaggcggctggcctgaaagtgcgccgtgtgaacaaggtgaccgaaggtcgccctcacgtggtcgacatgatcaagaacgacgaagtgtcgctgatcatcaacaccaccgaaggtcgccagtcgatcgccgactcctactcgattcgtcgcaatgcgctgcagcacaagatttactgcaccactaccattgcggctggtgaagccatctgcgaagcgctgaaattcggtccggaaaagaccgttcgtcgcttgcaggatctgcatgcaggactgaaagcatga

SEQ ID NO: 53 - protein, 1073 aa, Pseudomonas putida
MPKRTDIKSILILGAGPIVIGQACEFDYSGAQACKALREEGFRVILVNSNPATIMTDPAMADATYIEPIKWQSVAKIIEKERPDAVLPTMGGQTALNCALDLERHGVLEKFGVEMIGANADTIDKAEDRSRFDKAMKDIGLECPRSGIAHSMEEANAVLEKLGFPCIIRPSFTMGGTGGGIAYNREEFEEICTRGLDLSPTKELLIDESLIGWKEYEMEVVRDKKDNCIIVCSIENFDPMGVHTGDSITVAPAQTLTDKEYQIMRNASLAVLREIGVETGGSNVQFGICPNTGRMVVIEMNPRVSRSSALASKATGFPIAKIAAKLAIGYTLDELQNDITGGRTPASFEPSIDYVVTKLPRFAFEKFPKADARLTTQMKSVGEVMAIGRTFQESLQKALRGLEVGACGLDPKVDLASPEAASILKRELTVPGAERIWYVADAMRSGMTCEEIFNLTGIDMWFLVQMEDLIKEEEKVKTLALSAIDKDYMLRLKRKGFSDQRLAVLLGITDKNLRRHRHKLEVFPVYKRVDTCAAEFATDTAYLYSTYEEECEANPSTRDKIMILGGGPNRIGQGIEFDYCCVHAALALREDGYETIMVNCNPETVSTDYDTSDRLYFEPLTLEDVLEVCRVEKPKGVIVHYGGQTPLKLARALEEAGVPIIGTSPDAIDRAEDRERFQQMVQRLSLLQPPNATVRSEEEAIRAAGSIGYPLVVRPSYVLGGRAMEIVYELDELKRYLREAVQVSNDSPVLLDHFLNCAIEMDVDAVCDGTDVVIGAIMQHIEQAGVHSGDSACSLPPYSLSKEVQDEVRVQVKKMALELGVVGLMNVQLALQGDKIYVIEVNPRASRTVPFVSKCIGTSLAMIAARVMAGKTLKELGFTQEIIPNFYSVKEAVFPFAKFPGVDPILGPEMKSTGEVMGVGDSFGEAFAKAQMGASEVLPTGGTAFISVRDDDKPQVAGVARDLIALGFEVVATAGTAKVIEAAGLKVRRVNKVTEGRPHVVDMIKNDEVSLIINTTEGRQSIADSYSIRRNALQHKIYCTTTIAAGEAICEALKFGPEKTVRRLQDLHAGLKA

SEQ ID NO: 54 - DNA, 44 bp, synthetic oligonucleotide
agagcctgagcaaactggccgactgatgtggtgttggcttcttc

SEQ ID NO: 55 - DNA, 45 bp, synthetic oligonucleotide
ccgtgtgcttctcaaatgcctatttggtaatgctcatgctttcag

SEQ ID NO: 56 - DNA, 4841 bp, Pseudomonas putida
agagcctgagcaaactggccgactgatgtggtgttggcttcttcgcgggcttgcccgctcccacaggtgcggcgttgctcttgggctggtgcgatccctgtgggggcgcaccagcccgcgcagaagccaacacagatgtcagtctgtcgcattgatgtgttttagagacacatccgcggtagaccgaaaacacacttttctgtaagctacagctttagtgtgtccactaaaagcgcgcagcgaattgaattcagcacatgaaagcggggtgacgtgtccatacgtcactccgcttttttgcaacctgcgatcgccctttcatgcttgatttacgggaggtcttcttgacaaagccagccatactcgcccttgccgacggcagtattttccgcggtgaagccatcggtgccgacggtcagaccgttggtgaggtggtattcaacaccgctatgaccggctaccaggaaatccttacagacccttcctacgcgcagcaaatcgttaccctgacctacccgcacatcggcaacaccggtactaccccggaagacgccgagtcgagccgcgtctggtccgctggcctggtcatccgtgacctgccgctgctggccagcaactggcgtaacacccagtcgctgcctgagtacctcaaggccaacaacgtcgtcgccatcgccggcatcgacacccgtcgcctgacccgtatcctgcgtgaaaagggcgcccagaacggctgcattctggcgggtgacaacatcagcgaagaagctgccatcgctgctgcccgcggcttcccgggcctgaagggcatggacctggccaaggtcgtctccaccaaggaacgttacgagtggcgctccagcgtgtgggagctgaaaaccgacagccacccgaccatcgacgctgccgacctgccgtaccacgtggttgccttcgactatggcgtcaagctgaacatcctgcgcatgctggtggcccgcggctgccgcgtgaccgtggtaccagcccagaccccggccagcgaagtactggcactcaacccggacggcgtgttcctgtccaacggccctggtgaccctgagccgtgcgactacgcgatccaggcgatcaaggaaatcctcgaaaccgagatcccggtattcggcatctgcctcggccaccagctgctggccctggcgtccggcgccaagaccgtgaaaatgggccacggccaccacggtgccaaccacccggtccaggacctggatactggtgtggtcatgatcaccagccagaaccacggtttcgccgttgacgaggcgaccctgccgggcaacgttcgcgccattcacaagtcgctgttcgacggcaccctgcagggtatcgagcgtaccgacaagagcgcgttcagcttccagggccaccctgaagcgagcccgggcccgaccgacgtcgcgcctctgttcgatcgtttcaccgatgccatggccaagcgccgctgagcatcctgcttcaaggccccgggccggcacctgccgcgcccggcagcgcctgacccagattgttcaaagcggcttgccgactgaccccggatttgagtgaccaccatgccaaaacgtacagacatcaaaagcatcctgattctcggcgctggcccgatcgtgatcggccaggcctgcgaattcgactactccggcgcccaggcctgtaaagccctgcgcgaggaaggtttccgcgtcatcctggtgaactccaacccagccaccatcatgaccgacccggccatggctgacgccacctacatcgagccgatcaagtggcaatcggtggccaagatcatcgagaaagagcgcccggacgccgtcctgccgaccatgggtggccagaccgccctgaactgcgccctggacctggagcgccacggcgttctggagaagttcggcgtggagatgatcggtgccaacgctgacaccatcgacaaggccgaagaccgttcgcgcttcgacaaggccatgaaggacatcggcctggagtgcccgcgctccggtatcgcccacagcatggaagaggccaatgcggtcctcgagaagctcggcttcccgtgcatcattcgcccgtcgttcaccatgggcggcaccggcggcggtatcgcttacaaccgtgaagagttcgaagaaatctgcacccgtggtctggacctgtcgccgaccaaagagctgctgatcgacgaatcgctgatcggctggaaggaatacgagatggaggtggtccgcgacaagaaggacaactgcatcatcgtctgctcgatcgagaacttcgacccgatgggtgtgcacaccggtgactcgatcactgttgccccggcacagaccctgaccgacaaggaataccagatcatgcgcaacgcctcgctggcggtgctgcgtgaaatcggtgtggaaaccggcggttccaacgtccagttcggcatttgcccgaacaccggccgcatggttgtcatcgagatgaacccgcgcgtgtcgcgttcgtccgccctggcctccaaggccaccggcttcccgatcgccaagatcgccgccaagctggccattggttacaccctcgacgagctgcagaacgacatcactggcggtcgcaccccagcgtccttcgaaccttcgatcgactacgtcgtcaccaagctgccacgcttcgccttcgagaaattcccgaaagccgacgcccgcctgaccacccagatgaaatccgtgggtgaagtcatggccatcggccgtactttccaggaatccctgcagaaagccctgcgcggcctggaagtcggcgcctgcggcctcgacccgaaagtcgacctggccagcccggaagccgccagcatcctcaagcgcgaactgaccgtgccgggtgccgagcgtatctggtacgtggctgacgccatgcgttcgggcatgacctgcgaagaaatcttcaatctgaccggcatcgacatgtggttcctggtgcagatggaagacctgatcaaggaagaagagaaggtcaagaccctggccctgtcggcaatcgacaaggactacatgctgcgcctcaagcgcaagggcttctcggaccagcgcctggcagtactgctgggtatcaccgacaagaacctgcgtcgccaccgccacaagctggaagtgttcccggtgtacaagcgcgtcgacacctgcgccgccgagttcgccaccgacaccgcctacctgtactccacctacgaggaagagtgcgaggccaacccgtcgacccgcgacaagatcatgatcctgggtggcggcccgaaccgtatcggccaaggtatcgagttcgactactgctgcgtacacgccgccctggcgctgcgtgaagacggttacgagaccatcatggtcaactgcaacccggaaaccgtctccaccgactacgacacttccgaccgcctgtacttcgagccgctgaccctggaagacgtgctggaagtctgccgcgtcgagaagccgaagggcgtgatcgttcactacggcggccagaccccgctgaagctggcccgcgctctggaagaggctggcgtgccgatcatcggtaccagccctgacgccatcgaccgcgccgaagaccgcgagcgcttccagcagatggttcagcgcctgagcctgctgcagccgccaaacgccaccgtgcgcagcgaagaagaagccatccgtgctgcgggcagcatcggctacccgctggtcgtgcgtccgtcctacgtactgggcggccgtgccatggagatcgtctacgagctggacgagctcaagcgctacctgcgtgaagcggtacaagtgtcgaacgacagcccggtactgctcgaccacttcctcaactgcgccatcgagatggacgtggatgcggtgtgcgacggcaccgacgtggtcatcggcgcgatcatgcagcacatcgagcaggccggcgtacactccggcgactcggcgtgctcgctgccaccttactcgctgagcaaggaagtgcaggacgaagtccgcgttcaggtcaagaaaatggcgctggagctgggtgtagtcggcctgatgaacgtgcagctggccctgcagggcgacaagatctacgtgatcgaagtcaacccgcgtgcctcgcgtaccgtaccgttcgtgtccaagtgcatcggcacgtccctggcgatgatcgcagcccgtgtcatggcgggtaaaaccctgaaagagctgggcttcacccaggaaatcatcccgaacttctacagcgtgaaggaagccgtcttcccgttcgccaagttcccaggggttgacccgatcctcggccctgagatgaaatcgaccggtgaagtgatgggtgtcggtgacagcttcggtgaagccttcgccaaagcccagatgggtgccagcgaagtgctgccgactggcggtaccgcgttcatcagcgtgcgcgacgacgacaagccacaagtggccggcgttgcccgcgacctgatcgccctgggcttcgaagtggttgccactgccggcaccgccaaggttatcgaggcggctggcctgaaagtgcgccgtgtgaacaaggtgaccgaaggtcgccctcacgtggtcgacatgatcaagaacgacgaagtgtcgctgatcatcaacaccaccgaaggtcgccagtcgatcgccgactcctactcgattcgtcgcaatgcgctgcagcacaagatttactgcaccactaccattgcggctggtgaagccatctgcgaagcgctgaaattcggtccggaaaagaccgttcgtcgcttgcaggatctgcatgcaggactgaaagcatgagcattaccaaataggcatttgagaagcacacgg

SEQ ID NO: 57 - DNA, 18689 bp, various
tcaggcgggcaagaatgtgaataaaggccggataaaacttgtgcttatttttctttacggtctttaaaaaggccgtaatatccagctgaacggtctggttataggtacattgagcaactgactgaaatgcctcaaaatgttctttacgatgccattgggatatatcaacggtggtatatccagtgatttttttctccattttagcttccttagctcctgaaaatctcgataactcaaaaaatacgcccggtagtgatcttatttcattatggtgaaagttggaacctcttacgtgccgatcaacgtctcattttcgccaaaagttggcccagggcttcccggtatcaacagggacaccaggatttatttattctgcgaagtgatcttccgtcacaggtatttattcggcgcaaagtgcgtcgggtgatgctgccaacttactgatttagtgtatgatggtgtttttgaggtgctccagtggcttctgtttctatcagctgtccctcctgttcagctactgacggggtggtgcgtaacggcaaaagcaccgccggacatcagcgctagcggagtgtatactggcttactatgttggcactgatgagggtgtcagtgaagtgcttcatgtggcaggagaaaaaaggctgcaccggtgcgtcagcagaatatgtgatacaggatatattccgcttcctcgctcactgactcgctacgctcggtcgttcgactgcggcgagcggaaatggcttacgaacggggcggagatttcctggaagatgccaggaagatacttaacagggaagtgagagggccgcggcaaagccgtttttccataggctccgcccccctgacaagcatcacgaaatctgacgctcaaatcagtggtggcgaaacccgacaggactataaagataccaggcgtttccccctggcggctccctcgtgcgctctcctgttcctgcctttcggtttaccggtgtcattccgctgttatggccgcgtttgtctcattccacgcctgacactcagttccgggtaggcagttcgctccaagctggactgtatgcacgaaccccccgttcagtccgaccgctgcgccttatccggtaactatcgtcttgagtccaacccggaaagacatgcaaaagcaccactggcagcagccactggtaattgatttagaggagttagtcttgaagtcatgcgccggttaaggctaaactgaaaggacaagttttggtgactgcgctcctccaagccagttacctcggttcaaagagttggtagctcagagaaccttcgaaaaaccgccctgcaaggcggttttttcgttttcagagcaagagattacgcgcagaccaaaacgatctcaagaagatcatcttattaatcagataaaatatttctagatttcagtgcaatttatctcttcaaatgtagcacctgaagtcagccccatacgatataagttgtaattctcatgtttgacagcttatcatcgataagctttaatgcggtagtttatcacagttaaattgctaacgcagtcaggcaccgtgtatgaaatctaacaatgcgctcatcgtcatcctcggcaccgtcaccctggatgctgtaggcataggcttggttatgccggtactgccgggcctcttgcgggatatcgtccattccgacagcatcgccagtcactatggcgtgctgctagcgctatatgcgttgatgcaatttctatgcgcacccgttctcggagcactgtccgaccgctttggccgccgcccagtcctgctcgcttcgctacttggagccactatcgactacgcgatcatggcgaccacacccgtcctgtggatcctctacgccggacgcatcgtggccggcatcaccggcgccacaggtgcggttgctggcgcctatatcgccgacatcaccgatggggaagatcgggctcgccacttcgggctcatgagcgcttgtttcggcgtgggtatggtggcaggccccgtggccgggggactgttgggcgccatctccttgcatgcaccattccttgcggcggcggtgctcaacggcctcaacctactactgggctgcttcctaatgcaggagtcgcataagggagagcgtcgaccgatgcccttgagagccttcaacccagtcagctccttccggtgggcgcggggcatgactatcgtcgccgcacttatgactgtcttctttatcatgcaactcgtaggacaggtgccggcagcgctctgggtcattttcggcgaggaccgctttcgctggagcgcgacgatgatcggcctgtcgcttgcggtattcggaatcttgcacgccctcgctcaagccttcgtcactggtcccgccaccaaacgtttcggcgagaagcaggccattatcgccggcatggcggccgacgcgctgggctacgtcttgctggcgttcgcgacgcgaggctggatggccttccccattatgattcttctcgcttccggcggcatcgggatgcccgcgttgcaggccatgctgtccaggcaggtagatgacgaccatcagggacagcttcaaggatcgctcgcggctcttaccagcctaacttcgatcattggaccgctgatcgtcacggcgatttatgccgcctcggcgagcacatggaacgggttggcatggattgtaggcgccgccctataccttgtctgcctccccgcgttgcgtcgcggtgcatggagccgggccacctcgacctgaatggaagccggcggcacctcgctaacggattcaccactccaagaattggagccaatcaattcttgcggagaactgtgaatgcgcaaaccaacccttggcagaacatatccatcgcgtccgccatctccagcagccgcacgcggcgcatctcgggcagcgttgggtcctggccacgggtgcgcatgatcgtgctcctgtcgttgaggacccggctaggctggcggggttgccttactggttagcagaatgaatcaccgatacgcgagcgaacgtgaagcgactgctgctgcaaaacgtctgcgacctgagcaacaacatgaatggtcttcggtttccgtgtttcgtaaagtctggaaacgcggaagtcccctacgtgctgctgaagttgcccgcaacagagagtggaaccaaccggtgataccacgatactatgactgagagtcaacgccatgagcggcctcatttcttattctgagttacaacagtccgcaccgctgtccggtagctccttccggtgggcgcggggcatgactatcgtcgccgcacttatgactgtcttctttatcatgcaactcgtaggacaggtgccggcagcgcccaacagtcccccggccacggggcctgccaccatacccacgccgaaacaagcgccctgcaccattatgttccggatctgcatcgcaggatgctgctggctaccctgtggaacacctacatctgtattaacgaagcgctaaccgtttttatcaggctctgggaggcagaataaatgatcatatcgtcaattattacctccacggggagagcctgagcaaactggccgactgatgtggtgttggcttcttcgcgggcttgcccgctcccacaggtgcggcgttgctcttgggctggtgcgatccctgtgggggcgcaccagcccgcgcagaagccaacacagatgtcagtctgtcgcattgatgtgttttagagacacatccgcggtagaccgaaaacacacttttctgtaagctacagctttagtgtgtccactaaaagcgcgcagcgaattgaattcagcacatgaaagcggggtgacgtgtccatacgtcactccgcttttttgcaacctgcgatcgccctttcatgcttgatttacgggaggtcttcttgacaaagccagccatactcgcccttgccgacggcagtattttccgcggtgaagccatcggtgccgacggtcagaccgttggtgaggtggtattcaacaccgctatgaccggctaccaggaaatccttacagacccttcctacgcgcagcaaatcgttaccctgacctacccgcacatcggcaacaccggtactaccccggaagacgccgagtcgagccgcgtctggtccgctggcctggtcatccgtgacctgccgctgctggccagcaactggcgtaacacccagtcgctgcctgagtacctcaaggccaacaacgtcgtcgccatcgccggcatcgacacccgtcgcctgacccgtatcctgcgtgaaaagggcgcccagaacggctgcattctggcgggtgacaacatcagcgaagaagctgccatcgctgctgcccgcggcttcccgggcctgaagggcatggacctggccaaggtcgtctccaccaaggaacgttacgagtggcgctccagcgtgtgggagctgaaaaccgacagccacccgaccatcgacgctgccgacctgccgtaccacgtggttgccttcgactatggcgtcaagctgaacatcctgcgcatgctggtggcccgcggctgccgcgtgaccgtggtaccagcccagaccccggccagcgaagtactggcactcaacccggacggcgtgttcctgtccaacggccctggtgaccctgagccgtgcgactacgcgatccaggcgatcaaggaaatcctcgaaaccgagatcccggtattcggcatctgcctcggccaccagctgctggccctggcgtccggcgccaagaccgtgaaaatgggccacggccaccacggtgccaaccacccggtccaggacctggatactggtgtggtcatgatcaccagccagaaccacggtttcgccgttgacgaggcgaccctgccgggcaacgttcgcgccattcacaagtcgctgttcgacggcaccctgcagggtatcgagcgtaccgacaagagcgcgttcagcttccagggccaccctgaagcgagcccgggcccgaccgacgtcgcgcctctgttcgatcgtttcaccgatgccatggccaagcgccgctgagcatcctgcttcaaggccccgggccggcacctgccgcgcccggcagcgcctgacccagattgttcaaagcggcttgccgactgaccccggatttgagtgaccaccatgccaaaacgtacagacatcaaaagcatcctgattctcggcgctggcccgatcgtgatcggccaggcctgcgaattcgactactccggcgcccaggcctgtaaagccctgcgcgaggaaggtttccgcgtcatcctggtgaactccaacccagccaccatcatgaccgacccggccatggctgacgccacctacatcgagccgatcaagtggcaatcggtggccaagatcatcgagaaagagcgcccggacgccgtcctgccgaccatgggtggccagaccgccctgaactgcgccctggacctggagcgccacggcgttctggagaagttcggcgtggagatgatcggtgccaacgctgacaccatcgacaaggccgaagaccgttcgcgcttcgacaaggccatgaaggacatcggcctggagtgcccgcgctccggtatcgcccacagcatggaagaggccaatgcggtcctcgagaagctcggcttcccgtgcatcattcgcccgtcgttcaccatgggcggcaccggcggcggtatcgcttacaaccgtgaagagttcgaagaaatctgcacccgtggtctggacctgtcgccgaccaaagagctgctgatcgacgaatcgctgatcggctggaaggaatacgagatggaggtggtccgcgacaagaaggacaactgcatcatcgtctgctcgatcgagaacttcgacccgatgggtgtgcacaccggtgactcgatcactgttgccccggcacagaccctgaccgacaaggaataccagatcatgcgcaacgcctcgctggcggtgctgcgtgaaatcggtgtggaaaccggcggttccaacgtccagttcggcatttgcccgaacaccggccgcatggttgtcatcgagatgaacccgcgcgtgtcgcgttcgtccgccctggcctccaaggccaccggcttcccgatcgccaagatcgccgccaagctggccattggttacaccctcgacgagctgcagaacgacatcactggcggtcgcaccccagcgtccttcgaaccttcgatcgactacgtcgtcaccaagctgccacgcttcgccttcgagaaattcccgaaagccgacgcccgcctgaccacccagatgaaatccgtgggtgaagtcatggccatcggccgtactttccaggaatccctgcagaaagccctgcgcggcctggaagtcggcgcctgcggcctcgacccgaaagtcgacctggccagcccggaagccgccagcatcctcaagcgcgaactgaccgtgccgggtgccgagcgtatctggtacgtggctgacgccatgcgttcgggcatgacctgcgaagaaatcttcaatctgaccggcatcgacatgtggttcctggtgcagatggaagacctgatcaaggaagaagagaaggtcaagaccctggccctgtcggcaatcgacaaggactacatgctgcgcctcaagcgcaagggcttctcggaccagcgcctggcagtactgctgggtatcaccgacaagaacctgcgtcgccaccgccacaagctggaagtgttcccggtgtacaagcgcgtcgacacctgcgccgccgagttcgccaccgacaccgcctacctgtactccacctacgaggaagagtgcgaggccaacccgtcgacccgcgacaagatcatgatcctgggtggcggcccgaaccgtatcggccaaggtatcgagttcgactactgctgcgtacacgccgccctggcgctgcgtgaagacggttacgagaccatcatggtcaactgcaacccggaaaccgtctccaccgactacgacacttccgaccgcctgtacttcgagccgctgaccctggaagacgtgctggaagtctgccgcgtcgagaagccgaagggcgtgatcgttcactacggcggccagaccccgctgaagctggcccgcgctctggaagaggctggcgtgccgatcatcggtaccagccctgacgccatcgaccgcgccgaagaccgcgagcgcttccagcagatggttcagcgcctgagcctgctgcagccgccaaacgccaccgtgcgcagcgaagaagaagccatccgtgctgcgggcagcatcggctacccgctggtcgtgcgtccgtcctacgtactgggcggccgtgccatggagatcgtctacgagctggacgagctcaagcgctacctgcgtgaagcggtacaagtgtcgaacgacagcccggtactgctcgaccacttcctcaactgcgccatcgagatggacgtggatgcggtgtgcgacggcaccgacgtggtcatcggcgcgatcatgcagcacatcgagcaggccggcgtacactccggcgactcggcgtgctcgctgccaccttactcgctgagcaaggaagtgcaggacgaagtccgcgttcaggtcaagaaaatggcgctggagctgggtgtagtcggcctgatgaacgtgcagctggccctgcagggcgacaagatctacgtgatcgaagtcaacccgcgtgcctcgcgtaccgtaccgttcgtgtccaagtgcatcggcacgtccctggcgatgatcgcagcccgtgtcatggcgggtaaaaccctgaaagagctgggcttcacccaggaaatcatcccgaacttctacagcgtgaaggaagccgtcttcccgttcgccaagttcccaggggttgacccgatcctcggccctgagatgaaatcgaccggtgaagtgatgggtgtcggtgacagcttcggtgaagccttcgccaaagcccagatgggtgccagcgaagtgctgccgactggcggtaccgcgttcatcagcgtgcgcgacgacgacaagccacaagtggccggcgttgcccgcgacctgatcgccctgggcttcgaagtggttgccactgccggcaccgccaaggttatcgaggcggctggcctgaaagtgcgccgtgtgaacaaggtgaccgaaggtcgccctcacgtggtcgacatgatcaagaacgacgaagtgtcgctgatcatcaacaccaccgaaggtcgccagtcgatcgccgactcctactcgattcgtcgcaatgcgctgcagcacaagatttactgcaccactaccattgcggctggtgaagccatctgcgaagcgctgaaattcggtccggaaaagaccgttcgtcgcttgcaggatctgcatgcaggactgaaagcatgagcattaccaaataggcatttgagaagcacacggtcacactgcttccggtagtcaataaaccggtaaaccagcaatagacataagcggctatttaacgaccctgccctgaaccgacgaccgggtcgaatttgctttcgaatttctgccattcatccgcttattatcacttattcaggcgtagcaccaggcgtttaagggcaccaataactgccttaaaaaaattacgccccgccctgccactcatcgcagtactgttgtaattcattaagcattctgccgacatggaagccatcacaaacggcatgatgaacctgaatcgccagcggcatcagcaccttgtcgccttgcgtataatatttgcccatggatttaaatttaatctttctgcgaattgagatgacgccactggctgggcgtcatcccggtttcccgggtaaacaccaccgaaaaatagttactatcttcaaagccacattcggtcgaaatatcactgattaacaggcggctatgctggagaagatattgcgcatgacacactctgacctgtcgcagatattgattgatggtcattccagtctgctggcgaaattgctgacgcaaaacgcgctcactgcacgatgcctcatcacaaaatttatccagcgcaaagggacttttcaggctagccgccagccgggtaatcagcttatccagcaacgtttcgctggatgttggcggcaacgaatcactggtgtaacgatggcgattcagcaacatcaccaactgcccgaacagcaactcagccatttcgttagcaaacggcacatgctgactactttcatgctcaagctgaccgataacctgccgcgcctgcgccatccccatgctacctaagcgccagtgtggttgccctgcgctggcgttaaatcccggaatcgccccctgccagtcaagattcagcttcagacgctccgggcaataaataatattctgcaaaaccagatcgttaacggaagcgtaggagtgtttatcgtcagcatgaatgtaaaagagatcgccacgggtaatgcgataagggcgatcgttgagtacatgcaggccattaccgcgccagacaatcaccagctcacaaaaatcatgtgtatgttcagcaaagacatcttgcggataacggtcagccacagcgactgcctgctggtcgctggcaaaaaaatcatctttgagaagttttaactgatgcgccaccgtggctacctcggccagagaacgaagttgattattcgcaatatggcgtacaaatacgttgagaagattcgcgttattgcagaaagccatcccgtccctggcgaatatcacgcggtgaccagttaaactctcggcgaaaaagcgtcgaaaagtggttactgtcgctgaatccacagcgataggcgatgtcagtaacgctggcctcgctgtggcgtagcagatgtcgggctttcatcagtcgcaggcggttcaggtatcgctgaggcgtcagtcccgtttgctgcttaagctgccgatgtagcgtacgcagtgaaagagaaaattgatccgccacggcatcccaattcacctcatcggcaaaatggtcctccagccaggccagaagcaagttgagacgtgatgcgctgttttccaggttctcctgcaaactgcttttacgcagcaagagcagtaattgcataaacaagatctcgcgactggcggtcgagggtaaatcattttccccttcctgctgttccatctgtgcaaccagctgtcgcacctgctgcaatacgctgtggttaacgcgccagtgagacggatactgcccatccagctcttgtggcagcaactgattcagcccggcgagaaactgaaatcgatccggcgagcgatacagcacattggtcagacacagattatcggtatgttcatacagatgccgatcatgatcgcgtacgaaacagaccgtgccaccggtgatggtatagggctgcccattaaacacatgaatacccgtgccatgttcgacaatcacaatttcatgaaaatcatgatgatgttcaggaaaatccgcctgcgggagccggggttctatcgccacggacgcgttaccagacggaaaaaaatccacactatgtaatacggtcatactggcctcctgatgtcgtcaacacggcgaaatagtaatcacgaggtcaggttcttaccttaaattttcgacggaaaaccacgtaaaaaacgtcgatttttcaagatacagcgtgaattttcaggaaatgcggtgagcatcacatcaccacaattcagcaaattgtgaacatcatcacgttcatctttccctggttgccaatggcccattttcctgtcagtaacgagaaggtcgcgaattcaggcgctttttagactggtcgtaatgaacatttaaatgaattcccttgggactctagagatccgcgggggcccaggaggggggatctggcatttttgggaggtgtgaaatgagtgagaagatcgtcaactcgtggaacgaatgggatgagctcgaggagatggtggtcggcattgcggactatgccagcttcgaaccgaaagagccaggcaaccatcccaaactgcgcaaccagaacctggccgaaatcatccccttcccaagcggcccaaaggacccgaaggtgctggagaaagcgaacgaagagctgaatgggctggcttacctgctgaaggaccacgatgtgatcgtgcgtcgtcccgagaagatcgacttcaccaagagcctgaaaaccccgtatttcgaggttgccaaccagtactgcggcgtttgtcctcgcgacgtgatgatcacgtttggcaacgaaatcatggaagcgaccatgtccaaacgtgcacgcttcttcgaatacctcccctatcggaagctggtctacgagtactggaacaaggacgagcacatgatctggaacgcagccccgaaaccgaccatgcaggatagcatgtacctggaaaacttctgggagctctcgctggaagaacgcttcaagcggatgcacgacttcgaattctgcatcacccaagacgaggtgatcttcgatgccgccgattgctcccgcttgggtaaggacatcctggtgcaggaaagcatgaccaccaatcgcactggcatccgctggctgaagaagcatctcgaaccacgcggctttcgcgtccatccggtgcacttcccgttggacttcttccctagccacatcgactgcacgttcgtaccgttgcgtccgggtctgatcctgaccaatccggaacgcccgattcgcgaggaagaggagaagatcttcaaggagaatggctgggagctgatcaccgtaccgcagcctacctgctcgaacgacgagatgcccatgttctgccagagctcgaaatggctgtccatgaacgtcctgagcattagtcccaccaaggtgatctgcgaagaacgggaaaagccgctgcaagaactgctggacaagcacgggttcgaagtctttcccttgcctttccgccatgtgtttgagttcggtggcagctttcactgtgccacgtgggatattcgccgcaagggcgagtgcgaggactacctgccgaacctgaactaccagccgatttgcggctgacgcggatcccgacctgcataccgttgcagataaggtagtcactcatgagcgctaggcactttctctccctgctggacttcaccaccgacgaattgctcggggtgatccgccacggcatcgagctgaaggacctgcgcaagcgaggcgtgctgttcgaaccgctgaagaaccgtgtgctaggcatgatcttcgaaaagtcctcgacccgtacccgtgtgtcgttcgaggccggcatgatccagctcggcggccaggccatcttcctgtcgccccgcgacacccagctgggccgcggcgagccaattggtgacagcgccatcgtgctgtcgagcatggttgatgtggtgatgatccggacccacgcccacagcaccctgaccgagttcgccgccaagtcgcgtgtgcccgtgatcaacggcctgtccgacgaatcgcacccgtgccaactgctggccgacatgcagaccttcgttgaacaccgcggctcgattcagggcaagaccgtgacctggatcggcgatggcttcaacatgtgcaactcctatatcgaagccgccaggcagttcgatttccagctgcgcatcgcctgccccgaaggctatgagccggatcaacgcttcatggcactgggcggcgaccgcgtgcagatcatccgggatgccagggaagctgtgcgtgatgcacacctggtggtcaccgatgtctggacttccatgggtcaggaggaggaaactgcacggcgcctggcgcatttcgcgccttaccaggtcacccgcgaactgctcgacctggctgcacccgatgtcctcttcatgcactgcctgcccgcccaccgtggcgaggaaatcagccaggacctgctcgacgacccacgttcggtcgcctgggacgaggctgaaaaccgcctgcatgcacagaaggcgcttctcgaattccttgtagaaccggcttaccaccacgcatgagtcaaccgtacaaccccgtggagtgatggcatggcggacgtaaaaaaggtcgtactggcgtattccggcggccttgatacttcggtgattctcaagtggctgcaggatacctacaactgcgaagtggtgaccttcaccgctgacctggggcagggcgaagaggtcgaaccggcccgtgccaaggcccaggcaatgggcgttaaagagatctacatcgacgacctgcgcgaagaattcgtgcgtgatttcgtgttcccgatgttccgcgccaacaccgtctacgaaggcgagtacctgctgggtacttccatcgcccgtccgctgatcgccaagcgcctgatcgaaatcgccaacgaaaccggcgctgacgccatttcccatggcgccaccggcaagggtaacgaccaggtgcgcttcgagctgggtgcctatgccctgaagccaggcgtcaaggtcatcgctccatggcgcgagtgggacctgctgtcccgcgaaaagctgatggactacgccgagaagcacggcatcccgatcgagcgccacggcaagaagaagtcgccgtactcgatggacgccaacctgctgcacatctcctacgagggcggtgtcctggaagatacctggaccgagcacgaagaagacatgtggcgctggagtgtctcgcctgagaatgccccggaccaggctacctacatcgagctgacctaccgcaatggtgacatcgttgccatcgacggcgtcgagaaatccccggccaccgtcctggcagacctgaaccgtatcggtggtgccaacggcatcggccgtctggacatcgtcgaaaaccgttacgtcggcatgaagtcgcgcggttgctacgaaacgcctggcggtaccatcatgctcaaggcacaccgtgccatcgagtcgatcaccctggaccgcgaagtcgctcacctgaaagatgagctgatgccaaagtatgccagcctgatctacaccggctactggtggagcccggagcgtctgatgctgcaacagatgatcgatgcttcgcaggtcaacgtgaatggtgtggtgcgcctgaaactgtacaagggcaacgtgaccgtggttggccgcaagtcggacgattcgctgttcgatgccaacatcgccacctttgaagaagatggtggtgcctacaaccaggcagatgctgctggcttcatcaagctcaatgcactgcgtatgcgcattgccgccaacaagggccgttcgctgctctgattgctatcgacgccactttttcgttcacgcctgcaatgagtgaatccatgagcaccgagaagaccaatcagtcctggggcggccgcttcagtgagcccgtcgacgccttcgtcgcccgtttcaccgcctcggtagatttcgacaagcgcctgtaccgtcacgacatcatgggttcgattgcccatgccaccatgctggcgcaggtcggcgtgctcagtgatgccgagcgcgacaccatcatcgatggcctgaaaaccatccagggcgagattgaagccggcaacttcgactggcgtgtcgacctcgaagacgtgcacatgaacatcgaagcacgcctgaccgaccgcatcggcatcaccggcaagaagctgcatactgggcgtagccgcaacgaccaggtggccaccgacatccgcctttggctgcgcgacgaaatcgacctgatcctgggcgaaatcacccgcctgcagcagggcctgctggagcaggcagagcgtgaagccgaaaccatcatgcctggtttcacccacctgcagacggcgcagccggtcacctttggccaccacctgctggcgtggttcgaaatgctcagccgcgactatgagcgcctggtcgactgccgcaagcgcaccaaccgcatgccactgggcagcgccgcgctggccggcaccacctacccgatcgaccgtgaactgacctgcaagctgctgggctttgaagccgtggccggcaactcgctggatggcgtgtcggaccgtgatttcgccatcgaattctgcgccgctgccagcgtggcgatgatgcacctttcgcgcttctccgaagagctggtgctgtggaccagcgcgcagttccagttcatcgaccttccggaccgcttctgcactggcagctcgatcatgccgcagaaaaagaacccggacgtgccagagctggtacgtggcaagagcggccgcgtgttcggcgccctgaccggcctgctgaccctgatgaaaggccaaccgctggcctacaacaaggacaaccaggaagacaaggaaccgctgttcgacgccgccgataccctgcgcgactcgctgcgggccttcgctgacatgatcccggcgatcaagcccaagcacgccatcatgcgtgaagcggccctgcgcggtttctccaccgctaccgacctggctgactatctggttcgccgtggcctgccgttccgtgactgccacgagatcgttggccacgcggtgaagtatggtgtggacactggcaaggacctggccgagatgagcctggacgaactgcgccaattcagcgaccagatcgagcaggacgtgtttgccgtgctgacgctggaaggctcggtgaatgcgcgtgaccacattggtggtacggcgccggcgcaggtgcgtgctgccgtcgttcgtggcaaggccctgttggcgtctcgctaatcccccaaggctcgagcacgcgagagtagggaactgccaggcatcaaataaaacgaaaggctcagtcgaaagactgggcctttcgttttatctgttgtttgtcggtgaacgctctcctgagtaggacaaatccgccgggagcggatttgaacgatgataagctgtcaaacatgagaattcttgaagacgaaagggcctcgtgtgtacaaacgttcgtcaaaagggcgacacaaaattcctgcaggggccggcccagcgccggcggtcgagtggcgacggcgcggcttgtccgcgccctggtagattgcctggccgtaggccagccatttttgagcggccagcggccgcgataggccgacgcgaagcggcggggcgtagggagcgcagcgaccgaagggtaggcgctttttgcagctcttcggctgtgcgctggccagacagttatgcacaggccaggcgggttttaagagttttaataagttttaaagagttttaggcggaaaaatcgccttttttctcttttatatcagtcacttacatgtgtgaccggttcccaatgtacggctttgggttcccaatgtacgggttccggttcccaatgtacggctttgggttcccaatgtacgtgctatccacaggaaagagaccttttcgacctttttcccctgctagggcaatttgccctagcatctgctccgtacattaggaaccggcggatgcttcgccctcgatcaggttgcggtagcgcatgactaggatcgggccagcctgccccgcctcctccttcaaatcgtactccggcaggtcatttgacccgatcagcttgcgcacggtgaaacagaacttcttgaactctccggcgctgccactgcgttcgtagatcgtcttgaacaaccatctggcttctgccttgcctgcggcgcggcgtgccaggcggtagagaaaacggccgatgccgggatcgatcaaaaagtaatcggggtgaaccgtcagcacgtccgggttcttgccttctgtgatctcgcggtacatccaatcaactagctcgatctcgatgtactccggccgcccggtttcgctctttacgatcttgtagcggctaatcaaggcttcaccctcggataccgtcaccaggcggccgttcttggccttcttcgtacgctgcatggcaacgtgcgtggtgtttaaccgaatgcaggtttctaccaggtcgtctttctgctttccgccatcggctcgccggcagaacttgagtacgtccgcaacgtgtggacggaacacgcggccgggcttgtctcccttcccttcccggtatcggttcatggattcggttagatgggaaaccgccatcagtaccaggtcgtaatcccacacactggccatgccggccggccctgcggaaacctctacgtgcccgtctggaagctcgtagcggatcacctcgccagctcgtcggtcacgcttcgacagacggaaaacggccacgtccatgatgctgcgactatcgcgggtgcccacgtcatagagcatcggaacgaaaaaatctggttgctcgtcgcccttgggcggcttcctaatcgacggcgcaccggctgccggcggttgccgggattctttgcggattcgatcagcggccgcttgccacgattcaccggggcgtgcttctgcctcgatgcgttgccgctgggcggcctgcgcggccttcaacttctccaccaggtcatcacccagcgccgcgccgatttgtaccgggccggatggtttgcgaccgctcacgccgattcctcgggcttgggggttccagtgccattgcagggccggcagacaacccagccgcttacgcctggccaaccgcccgttcctccacacatggggcattccacggcgtcggtgcctggttgttcttgattttccatgccgcctcctttagccgctaaaattcatctactcatttattcatttgctcatttactctggtagctgcgcgatgtattcagatagcagctcggtaatggtcttgccttggcgtaccgcgtacatcttcagcttggtgtgatcctccgccggcaactgaaagttgacccgcttcatggctggcgtgtctgccaggctggccaacgttgcagccttgctgctgcgtgcgctcggacggccggcacttagcgtgtttgtgcttttgctcattttctctttacctcattaactcaaatgagttttgatttaatttcagcggccagcgcctggacctcgcgggcagcgtcgccctcgggttctgattcaagaacggttgtgccggcggcggcagtgcctgggtagctcacgcgctgcgtgatacgggactcaagaatgggcagctcgtacccggccagcgcctcggcaacctcaccgccgatgcgcgtgcctttgatcgcccgcgacacgacaaaggccgcttgtagccttccatccgtgacctcaatgcgctgcttaaccagctccaccaggtcggcggtggcccatatgtcgtaagggcttggctgcaccggaatcagcacgaagtcggctgccttgatcgcggacacagccaagtccgccgcctggggcgctccgtcgatcactacgaagtcgcgccggccgatggccttcacgtcgcggtcaatcgtcgggcggtcgatgccgacaacggttagcggttgatcttcccgcacggccgcccaatcgcgggcactgccctggggatcggaatcgactaacagaacatcggccccggcgagttgcagggcgcgggctagatgggttgcgatggtcgtcttgcctgacccgcctttctggttaagtacagcgataaccttcatgcgttccccttgcgtatttgtttatttactcatcgcatcatatacgcagcgaccgcatgacgcaagctgttttactcaaatacacatcacctttttagacggcggcgctcggtttcttcagcggccaagctggccggccaggccgccagcttggcatcagacaaaccggccaggatttcatgcagccgcacggttccggatgagcattca